European Patent Specification EP 3 628 011 B1, published August 5, 2026. Title: Gene Therapy For Ciliopathies. Applicant: UCL Business PLC. The sequence listing filed with the application follows.

SEQUENCE LISTING (49 sequences)

SEQ ID NO: 1 - DNA, 1782 bp, Homo sapiens
atggccgctgcgtcctcatcggattccgacgcctgcggagctgagagcaatgaggccaattcgaagtggttggatgcgcactacgacccaatggccaatatccacaccttttctgcctgcctagcgctggcagatttacatggggatggggaatacaagctggtggtaggggaccttggccctggtgggcagcagccccgcctgaaggtgctcaaaggaccactggtgatgaccgaaagcccgctacctgctctgccagctgctgctgccaccttcctcatggagcaacatgagccccggaccccagctctggcacttgcttcaggcccttgtgtctatgtgtataagaatctcagaccctacttcaagttcagcctgccccaattgcctccaaatcctctggaacaagacctttggaaccaggccaaagaggaccgaatcgaccccttaaccctgaaggagatgctggagagcatccgggagacggcagaggagcctttgtccatccagtcactcaggtttctgcagctggagctaagtgaaatggaggcatttgtaaaccaacacaagtccaactccatcaagcggcagacagtcatcaccaccatgaccaccttgaagaagaacctggctgacgaggatgctgtgtcttgcctggtgctgggcaccgagaacaaggagctcctggtgcttgaccccgaggccttcaccattttagccaagatgagccttcccagcgtccccgtcttcctagaggtttctggccagtttgatgttgagttccggcttgccgcggcctgccgcaatggaaacatctatattctgagaagagactccaagcaccccaagtactgcatcgagctgagcgcccagcctgtgggacttatccgggtacacaaggtcctagtggtgggcagcacccaagacagcctgcatggcttcacccacaaggggaagaagctgtggacagtgcagatgcccgcagccatcctgaccatgaacctcctggagcagcattcccggggcctgcaggccgtcatggctgggctggccaatggagaggtccgcatttatcgtgacaaggccctgctcaatgtcatccacaccccggatgcagtgaccagcctttgctttggccggtacgggcgggaggacaacaccctcatcatgaccactcgaggtggtggcctgatcatcaagatcctgaagcgtacagcagtgtttgtagagggaggaagtgaggtgggtcccccaccagcccaggccatgaaactcaatgtgccccgaaagacccggctttacgtggatcagacactgcgagagcgggaggctggcaccgccatgcaccgggccttccagacagacctatacctgctgcgcctacgtgctgcccgcgcctacctgcaggccctcgagtccagcctgagccccctgtccacgacagcccgagagccactcaagctgcacgccgtggttcagggccttggccccacctttaagctcacacttcacctgcagaacacctcaacaacccgtcctgtcctggggctgctggtctgcttcctgtacaacgaggcgctctattccctgccccgggccttcttcaaggtacccttgctggtgccagggctcaactaccccctggagacctttgtggagagtctcagtaacaagggcatctcagacatcatcaaggtgctggtgcttcgagaaggccaaagtgcacccctgctgagtgcccacgtcaacatgcctgggagcgaggggctggcggccgcctga

SEQ ID NO: 2 - DNA, 2172 bp, Homo sapiens
atgttaagttctatggccgctgcagggtctgtgaaggcggcgttgcaggtggccgaggtgctggaagccatcgtgagctgctgcgtggggcccgagggacggcaagttttgtgtacgaagcccactggcgaggtgcttctcagccggaatggaggccgcctcctggaggcgctacacttagagcatcccatagccaggatgatagtggactgtgtttccagtcatctcaaaaaaacaggagatggtgcaaaaacatttattatctttctttgccatttgcttagaggacttcatgcaatcacagacagagaaaaggatcctttgatgtgtgaaaacattcaaacccatggaaggcattggaaaaattgttctcggtggaaatttatttcccaggctctcctaacgtttcagacacaaatattagacggtattatggaccagtacctaagtagacactttttgtctatcttttcgtctgctaaagagagaacattgtgtaggagctctttagagttgctcttagaagcatacttttgtggaagagtgggaagaaataatcataaatttatttcacagttgatgtgtgactactttttcaagtgtatgacttgtaaaagtgggattggtgtatttgagttagtggatgaccattttgtagagttgaatgttggtgtcactggccttcctgtttcagattccaggatcatagctggtcttgtgcttcagaaagatttttctgtgtaccgcccagcagatggtgacatgcgaatggtgatagtaacagaaaccattcagcctcttttttccacttctggatcagagtttattctaaattcagaagcacagtttcagacatctcaattttggattatggaaaagacaaaagcaataatgaaacatctacatagtcagaatgtaaaattgctcatatctagtgtgaaacaaccagatttagttagttattatgcaggggtgaatggcatatcagtggttgagtgtttatcatcagaagaagtttctcttatccggaggatcattggtctttctccatttgtaccaccacaggccttttcgcagtgtgaaatacctaacactgctttggtgaaattttgtaaacctcttatccttagatccaaaagatatgttcatctaggcttgataagcacatgtgcatttataccacactctatagttctttgtggaccagtgcatggtctcattgaacaacatgaggatgctttacatggagcacttaaaatgcttcggcaattatttaaagaccttgatctaaattacatgacacaaaccaatgaccaaaatggcacttcaagtctttttatttataagaacagtggagaaagttatcaagcaccagatcctggtaatggctcaatacaaaggccttatcaggacacagttgcagagaacaaagatgcattggaaaaaactcaaacatatttaaaagtacattctaatttggtaattccagatgtagaattagaaacatatattccgtattcaacccccacactgacaccaacagatacattccaaacagttgaaacgctgacatgtttgtctttggaaagaaacaggctaactgattattatgaaccattactcaagaacaattccactgcttattcaacaaggggaaatagaatagaaatttcttacgaaaatttacaggtcacaaatattactagaaagggaagcatgttaccagtgagctgtaagttaccgaatatgggtacttcccagagttacctttcctcatctatgccagctggttgtgttttgccagtaggtggtaattttgagatcttgttacattactatcttctcaattatgccaaaaaatgccatcaatcagaagaaaccatggttagtatgataatagctaatgcacttttaggcattcccaaagtcctttataaatctaaaacaggaaagtacagctttccacatacatatataagagctgtccatgcactgcaaaccaatcaacccttggtaagcagtcagacaggtttggaatcagtaatgggtaaataccagctactaacttcagttcttcagtgtttgacaaaaatattaaccattgacatggtaatcactgttaagagacaccctcagaaagttcacaatcaagattcagaagatgaactataa

SEQ ID NO: 3 - DNA, 232 bp, Homo sapiens
ggctccggtgcccgtcagtgggcagagcgcacatcgcccacagtccccgagaagttggggggaggggtcggcaattgatccggtgcctagagaaggtggcgcggggtaaactgggaaagtgatgtcgtgtactggctccgcctttttcccgagggtgggggagaaccgtatataagtgcagtagtcgccgtgaacgttctttttcgcaacgggtttgccgccagaacacagg

SEQ ID NO: 4 - DNA, 584 bp, Artificial sequence
  CAG promoter sequence
gcgttacataacttacggtaaatggcccgcctggctgaccgcccaacgacccccgcccattgacgtcaataatgacgtatgttcccatagtaacgccaatagggactttccattgacgtcaatgggtggagtatttacggtaaactgcccacttggcagtacatcaagtgtatcatatgccaagtacgccccctattgacgtcaatgacggtaaatggcccgcctggcattatgcccagtacatgaccttatgggactttcctacttggcagtacatctacgtattagtcatcgctattaccatggtcgaggtgagccccacgttctgcttcactctccccatctcccccccctccccacccccaattttgtatttatttattttttaattattttgtgcagcgatgggggcggggggggggggggggcgcgcgccaggcggggcggggcggggcgaggggcggggcggggcgaggcggagaggtgcggcggcagccaatcagagcggcgcgctccgaaagtttccttttatggcgaggcggcggcggcggcggccctataaaaagcgaagcgcgcggcgggcg

SEQ ID NO: 5 - DNA, 1177 bp, Homo sapiens
ggtgcagcggcctccgcgccgggttttggcgcctcccgcgggcgcccccctcctcacggcgagcgctgccacgtcagacgaagggcgcaggagcgttcctgatccttccgcccggacgctcaggacagcggcccgctgctcataagactcggccttagaaccccagtatcagcagaaggacattttaggacgggacttgggtgactctagggcactggttttctttccagagagcggaacaggcgaggaaaagtagtcccttctcggcgattctgcggagggatctccgtggggcggtgaacgccgatgattatataaggacgcgccgggtgtggcacagctagttccgtcgcagccgggatttgggtcgcggttcttgtttgtggatcgctgtgatcgtcacttggtgagttgcgggctgctgggctggccggggctttcgtggccgccgggccgctcggtgggacggaagcgtgtggagagaccgccaagggctgtagtctgggtccgcgagcaaggttgccctgaactgggggttggggggagcgcacaaaatggcggctgttcccgagtcttgaatggaagacgcttgtaaggcgggctgtgaggtcgttgaaacaaggtggggggcatggtgggcggcaagaacccaaggtcttgaggccttcgctaatgcgggaaagctcttattcgggtgagatgggctggggcaccatctggggaccctgacgtgaagtttgtcactgactggagaactcgggtttgtcgtctggttgcgggggcggcagttatgcggtgccgttgggcagtgcacccgtacctttgggagcgcgcgcctcgtcgtgtcgtgacgtcacccgttctgttggcttataatgcagggtggggccacctgccggtaggtgtgcggtaggcttttctccgtcgcaggacgcagggttcgggcctagggtaggctctcctgaatcgacaggcgccggacctctggtgaggggagggataagtgaggcgtcagtttctttggtcggttttatgtacctatcttcttaagtagctgaagctccggttttgaactatgcgctcggggttggcgagtgtgttttgtgaagttttttaggcaccttttgaaatgtaatcatttgggtcaatatgtaattttcagtgttagactagtaaa

SEQ ID NO: 6 - DNA, 511 bp, Human cytomegalovirus
gatctgacggttcactaaacgagctctgcttatatagacctcccaccgtacacgcctaccgcccatttgcgtcaatggggcggagttgttacgacattttggaaagtcccgttgattttggtgccaaaacaaactcccattgacgtcaatggggtggagacttggaaatccccgtgagtcaaaccgctatccacgcccattgatgtactgccaaaaccgcatcaccatggtaatagcgatgactaatacgtagatgtactgccaagtaggaaagtcccataaggtcatgtactgggcataatgccaggcgggccatttaccgtcattgacgtcaatagggggcgtacttggcatatgatacacttgatgtactgccaagtgggcagtttaccgtaaatactccacccattgacgtcaatggaaagtccctattggtcattattgacgtcaatgggcgggggtcgttgggcggtcagccaggcgggccatttaccgtaagttatgtaacggg

SEQ ID NO: 7 - DNA, 511 bp, Mus musculus
ttctaccgggtaggggaggcgcttttcccaaggcagtctggagcatgcgctttagcagccccgctgggcacttggcgctacacaagtggcctctggcctcgcacacattccacatccaccggtaggcgccaaccggctccgttctttggtggccccttcgcgccaccttctactcctcccctagtcaggaagttcccccccgccccgcagctcgcgtcgtgcaggacgtgacaaatggaagtagcacgtctcactagtctcgtgcagatggacagcaccgctgagcaatggaagcgggtaggcctttggggcagcggccaatagcagctttgctccttcgctttctgggctcagaggctgggaaggggtgggtccgggggcgggctcaggggcgggctcaggggcggggcgggcgcccgaaggtcctccggaggcccggcattctgcacgcttcaaaagcgcacgtctgccgcgctgttctcctcttcctcatctccgggcctttcgacct

SEQ ID NO: 8 - DNA, 260 bp, Gallus gallus
cacgttctgcttcactctccccatctcccccccctccccacccccaattttgtatttatttattttttaattattttgtgcagcgatgggggcggggggggggggggcgcgcgccaggcggggcggggcggggcgaggggcggggcggggcgaggcggagaggtgcggcggcagccaatcagagcggcgcgctccgaaagtttccttttatggcgaggcggcggcggcggcggccctataaaaagcgaagcgcgcggcgg

SEQ ID NO: 9 - protein, 593 aa, Homo sapiens
MAAASSSDSDACGAESNEANSKWLDAHYDPMANIHTFSACLALADLHGDGEYKLVVGDLGPGGQQPRLKVLKGPLVMTESPLPALPAAAATFLMEQHEPRTPALALASGPCVYVYKNLRPYFKFSLPQLPPNPLEQDLWNQAKEDRIDPLTLKEMLESIRETAEEPLSIQSLRFLQLELSEMEAFVNQHKSNSIKRQTVITTMTTLKKNLADEDAVSCLVLGTENKELLVLDPEAFTILAKMSLPSVPVFLEVSGQFDVEFRLAAACRNGNIYILRRDSKHPKYCIELSAQPVGLIRVHKVLVVGSTQDSLHGFTHKGKKLWTVQMPAAILTMNLLEQHSRGLQAVMAGLANGEVRIYRDKALLNVIHTPDAVTSLCFGRYGREDNTLIMTTRGGGLIIKILKRTAVFVEGGSEVGPPPAQAMKLNVPRKTRLYVDQTLREREAGTAMHRAFQTDLYLLRLRAARAYLQALESSLSPLSTTAREPLKLHAVVQGLGPTFKLTLHLQNTSTTRPVLGLLVCFLYNEALYSLPRAFFKVPLLVPGLNYPLETFVESLSNKGISDIIKVLVLREGQSAPLLSAHVNMPGSEGLAAA

SEQ ID NO: 10 - protein, 723 aa, Homo sapiens
MLSSMAAAGSVKAALQVAEVLEAIVSCCVGPEGRQVLCTKPTGEVLLSRNGGRLLEALHLEHPIARMIVDCVSSHLKKTGDGAKTFIIFLCHLLRGLHAITDREKDPLMCENIQTHGRHWKNCSRWKFISQALLTFQTQILDGIMDQYLSRHFLSIFSSAKERTLCRSSLELLLEAYFCGRVGRNNHKFISQLMCDYFFKCMTCKSGIGVFELVDDHFVELNVGVTGLPVSDSRIIAGLVLQKDFSVYRPADGDMRMVIVTETIQPLFSTSGSEFILNSEAQFQTSQFWIMEKTKAIMKHLHSQNVKLLISSVKQPDLVSYYAGVNGISVVECLSSEEVSLIRRIIGLSPFVPPQAFSQCEIPNTALVKFCKPLILRSKRYVHLGLISTCAFIPHSIVLCGPVHGLIEQHEDALHGALKMLRQLFKDLDLNYMTQTNDQNGTSSLFIYKNSGESYQAPDPGNGSIQRPYQDTVAENKDALEKTQTYLKVHSNLVIPDVELETYIPYSTPTLTPTDTFQTVETLTCLSLERNRLTDYYEPLLKNNSTAYSTRGNRIEISYENLQVTNITRKGSMLPVSCKLPNMGTSQSYLSSSMPAGCVLPVGGNFEILLHYYLLNYAKKCHQSEETMVSMIIANALLGIPKVLYKSKTGKYSFPHTYIRAVHALQTNQPLVSSQTGLESVMGKYQLLTSVLQCLTKILTIDMVITVKRHPQKVHNQDSEDEL

SEQ ID NO: 11 - DNA, 1782 bp, Artificial sequence
  Codon optimised nucleotide sequence encoding human BBS1 protein (referred to as COSEQ1-BBS1)
atggctgccgccagcagttctgattctgatgcctgtggcgccgagagcaacgaggccaattctaaatggctggacgcccactacgaccccatggccaatatccacacctttagcgcctgtctggccctggctgatcttcatggcgacggcgagtataagctggttgtgggagatcttggacctggcggacagcagcctagactgaaggtgctgaagggccctctcgtgatgacagagtctcctcttcctgctctgcctgccgccgctgccacatttctgatggaacagcacgagcccagaacacccgctctggctcttgcttctggcccttgcgtgtacgtgtacaagaacctgcggccttacttcaagttcagcctgcctcagctgcctcctaatcctctggaacaggacctgtggaaccaggccaaagaggacagaatcgaccctctgacactgaaagagatgctggaatccatcagagagacagccgaggaacccctgtctatccagagcctgagattcctgcagctggaactgagcgagatggaagccttcgtgaaccagcacaagagcaacagcatcaagcggcagaccgtgatcaccaccatgaccacactgaagaagaacctggccgacgaggatgccgtgtcttgtctggtgctgggcaccgagaacaaagagctgctggttctggatcccgaggccttcacaatcctggccaagatgtctctgcctagcgtgcccgtgtttctggaagtgtccggccagttcgacgtggaatttcggctggccgctgcctgcagaaacggcaacatctacatcctgcggagggacagcaagcaccccaagtactgtatcgagctgtctgcccagcctgtgggcctgattagagtgcacaaggtgctggtcgtgggcagcacacaggatagcctgcacggctttacccacaagggcaagaaactgtggaccgtgcagatgccagccgccatcctgaccatgaatctgctcgaacagcacagcagaggactgcaggctgttatggcaggactggctaatggcgaagtgcggatctacagagacaaggccctgctgaacgtgatccacacacctgatgccgtgacaagcctgtgcttcggcagatacggcagagaggacaacaccctgatcatgacaacaagaggcggcggactgatcatcaagatcctgaagagaaccgccgtgttcgtggaaggcggatctgaagttggacctcctccagctcaggccatgaagctgaatgtgcccagaaagacccggctgtacgtggaccagacactgagagaaagagaagccggcacagccatgcacagagccttccagactgacctgtacctgctgagactgagagccgccagagcctatctgcaggccctggaatctagcctgtctcctctgagcacaaccgccagagagcctctgaaactgcacgctgtggttcaaggcctgggacctaccttcaagctgaccctgcatctgcagaacaccagcaccacaagaccagtgctgggcctgctcgtgtgcttcctgtacaatgaggccctgtacagcctgccacgggccttttttaaggtgccactgctggtgcccggcctgaactaccctctggaaacctttgtggaaagcctgagcaacaagggcatcagcgacatcatcaaagtgctggtgctgagagagggccagtctgctcctctgctcagcgcccatgtgaatatgcctggctctgaaggcctggcagccgcttaa

SEQ ID NO: 12 - DNA, 1782 bp, Artificial sequence
  Codon optimised nucleotide sequence encoding human BBS1 protein (referred to as COSEQ2-BBS1)
atggctgccgcctctagctctgactctgatgcatgtggagcagagtctaacgaggccaatagcaagtggctggacgcccactacgatcctatggccaacatccacacattctctgcctgcctggccctggcagacctgcacggcgatggagagtataagctggtggtgggcgacctgggacctggcggccagcagccacggctgaaggtgctgaagggccctctggtcatgacagagtccccactgcccgccctgccagccgccgccgccaccttcctgatggagcagcacgagcctagaaccccagccctggccctggcctctggcccctgcgtgtacgtgtataagaacctgcggccctacttcaagtttagcctgccacagctgccccctaaccctctggagcaggatctgtggaatcaggccaaggaggacaggatcgatcctctgacactgaaggagatgctggagagcatccgggagacagccgaggagccactgagcatccagtccctgagattcctgcagctggagctgtccgagatggaggcctttgtgaaccagcacaagtctaatagcatcaagcgccagaccgtgatcaccacaatgaccacactgaagaagaacctggccgacgaggatgccgtgtcttgtctggtgctgggcacagagaataaggagctgctggtgctggacccagaggccttcaccatcctggccaagatgtctctgccctctgtgcccgtgttcctggaggtgagcggacagttcgacgtggagtttcggctggctgccgcctgcagaaacggcaatatctacatcctgcggagagatagcaagcacccaaagtattgtattgagctgtccgcccagcctgtgggcctgatcagagtgcacaaggtgctggtggtgggcagcacccaggactccctgcacggcttcacacacaagggcaagaagctgtggaccgtgcagatgcccgccgccatcctgaccatgaacctgctggagcagcacagcagaggcctgcaggccgtgatggcaggcctggcaaatggagaggtgaggatctaccgcgacaaggccctgctgaatgtgatccacacccctgatgccgtgacatccctgtgcttcggccggtatggcagagaggataacacactgatcatgaccacacggggcggcggcctgatcatcaagatcctgaagagaacagccgtgtttgtggagggcggctctgaagtgggcccaccccctgcccaggccatgaagctgaatgtgcccaggaagacccgcctgtacgtggaccagacactgagggaaagagaggcaggaacagcaatgcacagggccttccagaccgatctgtacctgctgagactgagagcagcaagagcctatctgcaggccctggagagctccctgtccccactgtctaccacagcaagagaacccctgaagctgcacgcagtggtgcagggcctgggacccaccttcaagctgacactgcacctgcagaacacatccaccacaaggcctgtgctgggcctgctggtgtgcttcctgtacaatgaggccctgtattctctgccacgcgccttctttaaggtgccactgctggtgcccggcctgaactatcccctggagacattcgtggagtccctgtctaataagggcatctctgatatcatcaaggtgctggtgctgagagaaggacagtccgcccctctgctgtctgcccacgtgaatatgccaggcagcgagggcctggctgccgcctga

SEQ ID NO: 13 - DNA, 2172 bp, Artificial sequence
  Codon optimised nucleotide sequence encoding human BBS10 protein (referred to as COSEQ1-BBS10)
atgctgtctagcatggctgccgctggatctgtgaaagctgctctgcaggttgccgaggtgctggaagccatcgtgtcttgttgtgtgggacctgagggcagacaggtgctgtgtacaaagcctacaggcgaagtgctgctgagcagaaatggcggcagactgctcgaagccctgcacctggaacaccctatcgccagaatgatcgtggactgcgtgtccagccacctgaagaaaacaggcgacggcgccaagaccttcatcatctttctgtgccatctgctgcggggcctgcacgccatcaccgatagagaaaaggaccctctgatgtgcgagaacatccagacacacggccggcactggaagaactgctcccggtggaagtttatcagccaggctctgctgacctttcagacccagatcctggacggcatcatggaccagtacctgagcagacacttcctgagcatcttcagcagcgccaaagaacggaccctgtgcagaagctctctggaactgctgctcgaggcctacttttgcggcagagtgggcagaaacaaccacaagttcatctcccagctgatgtgtgactacttcttcaagtgcatgacctgcaagagcggcatcggcgtgttcgagctggtggacgatcacttcgtggaactgaatgtgggcgtgaccggcctgcctgtgtccgatagcagaattattgccggcctggtgctgcagaaagacttcagcgtgtacagacccgccgacggcgacatgagaatggtcatcgtgaccgagacaatccagcctctgttcagcacaagcggcagcgagttcatcctgaacagcgaggcccagtttcagaccagccagttctggatcatggaaaagaccaaggccatcatgaagcacctccacagccagaacgtgaagctgctgatctccagcgtgaagcagcccgacctggtgtcttattatgccggcgtgaacggcatcagcgtggtggaatgtctgagcagcgaagaggtgtccctgatcagacggatcatcggactgagcccctttgtgcctcctcaagcctttagccagtgcgagatccctaacacagccctggtcaagttctgcaagcccctgatcctgcggagcaagagatatgtgcacctgggcctgatcagcacatgcgccttcattcctcactccatcgtgctgtgtggacctgtgcacggactgattgagcagcacgaagatgcactgcacggcgccctgaaaatgctgagacagctgttcaaggacctggacctgaactacatgacccagaccaacgaccagaacggcaccagcagcctgttcatctacaagaacagcggcgagagctatcaggccccagatccaggcaatggcagcatccagaggccttaccaggataccgtggccgagaacaaggacgccctggaaaaaacccagacctacctgaaggtgcacagcaacctggtcatccccgatgtggaactggaaacctacattccctacagcacccctacactgacccctaccgataccttccagaccgtggaaaccctgacctgtctgagcctggaacggaacagactgaccgactactacgagcccctgctgaaaaacaacagcaccgcctatagcacccggggcaacagaatcgagatcagctacgagaacctgcaagtgaccaacatcacccggaagggctccatgctgccagtgtcctgcaagctgcctaatatgggcaccagccagagctacctgtcctcttctatgcctgccggatgtgtgctgcctgtcggcggcaattttgagatcctgctgcactactacctgctgaactacgccaagaagtgccaccagagcgaagagacaatggtgtccatgattatcgccaacgctctgctgggcatccccaaggtgctgtacaagagcaagaccggcaagtacagcttccctcacacctacattagagccgtgcacgccctgcagaccaatcagccactggtttctagccagacaggcctggaaagcgtgatgggaaagtaccagctgctgaccagcgtgctgcagtgcctgaccaagatcctgaccatcgacatggtcatcaccgtgaagcggcaccctcagaaagtgcacaaccaggacagcgaggacgagctgtag

SEQ ID NO: 14 - DNA, 2172 bp, Artificial sequence
  Codon optimised nucleotide sequence encoding human BBS10 protein (referred to as COSEQ2-BBS10)
atgctgagctccatggctgccgccggatctgtgaaagccgccctgcaggtggcagaggtgctggaggcaatcgtgagctgttgcgtgggacctgagggccggcaggtgctgtgcacaaagccaaccggcgaggtgctgctgtctagaaatggcggccggctgctggaggccctgcacctggagcacccaattgcaagaatgatcgtggactgcgtgtctagccacctgaagaagacaggcgatggcgccaagaccttcatcatcttcctgtgccacctgctgaggggcctgcacgccatcacagaccgcgagaaggatcctctgatgtgcgagaacatccagacccacggcaggcactggaagaattgttcccgctggaagttcatctctcaggccctgctgacatttcagacccagatcctggacggcatcatggatcagtatctgagcaggcacttcctgtccatcttttcctctgccaaggagcggaccctgtgcagaagctccctggagctgctgctggaggcctacttctgtggccgggtgggcagaaacaatcacaagtttatcagccagctgatgtgcgactatttctttaagtgcatgacctgtaagtccggcatcggcgtgttcgagctggtggacgatcactttgtggagctgaacgtgggagtgacaggcctgcccgtgtccgactctcgcatcatcgccggcctggtgctgcagaaggatttctccgtgtaccggcctgccgacggcgatatgagaatggtcatcgtgaccgagacaatccagccactgttcagcacctccggctctgagttcatcctgaacagcgaggcccagttccagacatctcagttttggatcatggagaagaccaaggccatcatgaagcacctgcacagccagaacgtgaagctgctgatctctagcgtgaagcagccagacctggtgtcttactatgccggcgtgaatggcatcagcgtggtggagtgtctgtcctctgaggaggtgtccctgatccggagaatcattggcctgtctcccttcgtgccccctcaggcctttagccagtgcgagatccccaacacagccctggtgaagttctgtaagcctctgatcctgaggtccaagcggtacgtgcacctgggcctgatcagcacctgcgcctttatcccacactctatcgtgctgtgcggacctgtgcacggcctgattgagcagcacgaggatgcactgcacggcgccctgaagatgctgaggcagctgttcaaggacctggatctgaattacatgacccagacaaacgaccagaatggcacaagctccctgtttatctacaagaactctggcgagagctatcaggccccagatcccggcaatggcagcattcagcgcccctaccaggacacagtggcagagaacaaggatgccctggagaagacccagacatatctgaaggtgcactccaacctggtcatccctgacgtggagctggagacatacatcccttattctaccccaacactgacccccacagataccttccagacagtggagacactgacctgcctgtccctggagaggaaccgcctgaccgactactatgagcccctgctgaagaacaattccacagcctactctacccggggcaatagaatcgagatcagctatgagaacctgcaggtgacaaatatcaccagaaagggctctatgctgcctgtgagctgcaagctgccaaacatgggcaccagccagtcctacctgtctagctccatgcctgcaggatgcgtgctgcctgtgggcggcaacttcgagatcctgctgcactactatctgctgaattatgccaagaagtgccaccagagcgaggagacaatggtgtccatgatcatcgccaacgccctgctgggcatcccaaaggtgctgtacaagtctaagaccggcaagtacagctttccccacacctatatccgggccgtgcacgccctgcagacaaatcagcctctggtgtctagccagaccggcctggagtccgtgatgggcaagtaccagctgctgacatctgtgctgcagtgtctgacaaagatcctgaccatcgatatggtcatcaccgtgaagagacacccacagaaggtgcacaatcaggacagcgaggatgagctgtaa

SEQ ID NO: 15 - DNA, 3030 bp, Artificial sequence
  Construct comprising EFS promoter and wild type BBS1 nucleotide sequence (referred to as EFS-WTBBS1)
actagtgggcagatctcgatcgagttgggccccagagcttggctccggtgcccgtcagtgggcagagcgcacatcgcccacagtccccgagaagttgtggggaggggtcggcaattgaaccggtgcctagagaaggtggcgcggggtaaactgggaaagtgatgtcgtgtactggctccgcctttttcccgagggtgggggagaaccgtatataagtgcagtagtcgccgtgaacgttctttttcgcaacgggtttgccgccagaacacaggtaagtgccgtgtgtggttcccgcgggcctggcctctttacgggttatggcccttgcgtgccttgaattactccacctggctgcagtacgtgattcttgatcccgagcttcgggttggaagtgggtgggagagttcgaggccttgcgcttaaggagccccttcgcctcgtgcttgagttgaggcctggcctgggcgctggggccgccgcgtgcgaatctggtggcaccttcgcgcctgtctcgctgctttcgataagtctctagccatttaaaatttttgatgacctgctgcgacgctttttttctggcaagatagtcttgtaaatgcgggccaagatctgcacactggtatttcggtttttggggccgcgggcggcgacggggcccgtgcgtcccagcgcacatgttcggcgaggcggggcctgcgagcgcggccaccgagaatcggacgggggtagtctcaagctggccggcctgctctggtgcctggcctcgcgccgccgtgtatcgccccgccctgggcggcaaggctggcccggtcggcaccagttgcgtgagcggaaagatggccgcttcccggccctgctgcagggagctcaaaatggaggacgcggcgctcgggagagcgggcgggtgagtcacccacacaaaggaaaagggcctttccgtcctcagccgtcgcttcatgtgactccacggagtaccgggcgccgtccaggcacctcgattagttctcgagcttttggagtacgtcgtctttaggttggggggaggggttttatgcgatggagtttccccacactgagtgggtggagactgaagttaggccagcttggcacttgatgtaattctccttggaatttgccctttttgagtttggatcttggttcattctcaagcctcagacagtggttcaaagtttttttcttccatttcaggtgtcgtgaccatgagcttcgaattccgatggccgctgcgtcctcatcggattccgacgcctgcggagctgagagcaatgaggccaattcgaagtggttggatgcgcactacgacccaatggccaatatccacaccttttctgcctgcctagcgctggcagatttacatggggatggggaatacaagctggtggtaggggaccttggccctggtgggcagcagccccgcctgaaggtgctcaaaggaccactggtgatgaccgaaagcccgctacctgctctgccagctgctgctgccaccttcctcatggagcaacatgagccccggaccccagctctggcacttgcttcaggcccttgtgtctatgtgtataagaatctcagaccctacttcaagttcagcctgccccaattgcctccaaatcctctggaacaagacctttggaaccaggccaaagaggaccgaatcgaccccttaaccctgaaggagatgctggagagcatccgggagacggcagaggagcctttgtccatccagtcactcaggtttctgcagctggagctaagtgaaatggaggcatttgtaaaccaacacaagtccaactccatcaagcggcagacagtcatcaccaccatgaccaccttgaagaagaacctggctgacgaggatgctgtgtcttgcctggtgctgggcaccgagaacaaggagctcctggtgcttgaccccgaggccttcaccattttagccaagatgagccttcccagcgtccccgtcttcctagaggtttctggccagtttgatgttgagttccggcttgccgcggcctgccgcaatggaaacatctatattctgagaagagactccaagcaccccaagtactgcatcgagctgagcgcccagcctgtgggacttatccgggtacacaaggtcctagtggtgggcagcacccaagacagcctgcatggcttcacccacaaggggaagaagctgtggacagtgcagatgcccgcagccatcctgaccatgaacctcctggagcagcattcccggggcctgcaggccgtcatggctgggctggccaatggagaggtccgcatttatcgtgacaaggccctgctcaatgtcatccacaccccggatgcagtgaccagcctttgctttggccggtacgggcgggaggacaacaccctcatcatgaccactcgaggtggtggcctgatcatcaagatcctgaagcgtacagcagtgtttgtagagggaggaagtgaggtgggtcccccaccagcccaggccatgaaactcaatgtgccccgaaagacccggctttacgtggatcagacactgcgagagcgggaggctggcaccgccatgcaccgggccttccagacagacctatacctgctgcgcctacgtgctgcccgcgcctacctgcaggccctcgagtccagcctgagccccctgtccacgacagcccgagagccactcaagctgcacgccgtggttcagggccttggccccacctttaagctcacacttcacctgcagaacacctcaacaacccgtcctgtcctggggctgctggtctgcttcctgtacaacgaggcgctctattccctgccccgggccttcttcaaggtacccttgctggtgccagggctcaactaccccctggagacctttgtggagagtctcagtaacaagggcatctcagacatcatcaaggtgctggtgcttcgagaaggccaaagtgcacccctgctgagtgcccacgtcaacatgcctgggagcgaggggctggcggccgcctgagacttgtcgac

SEQ ID NO: 16 - DNA, 3035 bp, Artificial sequence
  Construct comprising EFS promoter and COSEQ1-BBS1 nucleotide sequence (referred to as EFS-COSEQ1-BBS1)
actagtgggcagatctcgatcgagttgggccccagagcttggctccggtgcccgtcagtgggcagagcgcacatcgcccacagtccccgagaagttgtggggaggggtcggcaattgaaccggtgcctagagaaggtggcgcggggtaaactgggaaagtgatgtcgtgtactggctccgcctttttcccgagggtgggggagaaccgtatataagtgcagtagtcgccgtgaacgttctttttcgcaacgggtttgccgccagaacacaggtaagtgccgtgtgtggttcccgcgggcctggcctctttacgggttatggcccttgcgtgccttgaattacttccacctggctgcagtacgtgattcttgatcccgagcttcgggttggaagtgggtgggagagttcgaggccttgcgcttaaggagccccttcgcctcgtgcttgagttgaggcctggcctgggcgctggggccgccgcgtgcgaatctggtggcaccttcgcgcctgtctcgctgctttcgataagtctctagccatttaaaatttttgatgacctgctgcgacgctttttttctggcaagatagtcttgtaaatgcgggccaagatctgcacactggtatttcggtttttggggccgcgggcggcgacggggcccgtgcgtcccagcgcacatgttcggcgaggcggggcctgcgagcgcggccaccgagaatcggacgggggtagtctcaagctggccggcctgctctggtgcctggcctcgcgccgccgtgtatcgccccgccctgggcggcaaggctggcccggtcggcaccagttgcgtgagcggaaagatggccgcttcccggccctgctgcagggagctcaaaatggaggacgcggcgctcgggagagcgggcgggtgagtcacccacacaaaggaaaagggcctttccgtcctcagccgtcgcttcatgtgactccacggagtaccgggcgccgtccaggcacctcgattagttctcgagcttttggagtacgtcgtctttaggttggggggaggggttttatgcgatggagtttccccacactgagtgggtggagactgaagttaggccagcttggcacttgatgtaattctccttggaatttgccctttttgagtttggatcttggttcattctcaagcctcagacagtggttcaaagtttttttcttccatttcaggtgtcgtgaccatgagcttcgaattcgccaccatggctgccgccagcagttctgattctgatgcctgtggcgccgagagcaacgaggccaattctaaatggctggacgcccactacgaccccatggccaatatccacacctttagcgcctgtctggccctggctgatcttcatggcgacggcgagtataagctggttgtgggagatcttggacctggcggacagcagcctagactgaaggtgctgaagggccctctcgtgatgacagagtctcctcttcctgctctgcctgccgccgctgccacatttctgatggaacagcacgagcccagaacacccgctctggctcttgcttctggcccttgcgtgtacgtgtacaagaacctgcggccttacttcaagttcagcctgcctcagctgcctcctaatcctctggaacaggacctgtggaaccaggccaaagaggacagaatcgaccctctgacactgaaagagatgctggaatccatcagagagacagccgaggaacccctgtctatccagagcctgagattcctgcagctggaactgagcgagatggaagccttcgtgaaccagcacaagagcaacagcatcaagcggcagaccgtgatcaccaccatgaccacactgaagaagaacctggccgacgaggatgccgtgtcttgtctggtgctgggcaccgagaacaaagagctgctggttctggatcccgaggccttcacaatcctggccaagatgtctctgcctagcgtgcccgtgtttctggaagtgtccggccagttcgacgtggaatttcggctggccgctgcctgcagaaacggcaacatctacatcctgcggagggacagcaagcaccccaagtactgtatcgagctgtctgcccagcctgtgggcctgattagagtgcacaaggtgctggtcgtgggcagcacacaggatagcctgcacggctttacccacaagggcaagaaactgtggaccgtgcagatgccagccgccatcctgaccatgaatctgctcgaacagcacagcagaggactgcaggctgttatggcaggactggctaatggcgaagtgcggatctacagagacaaggccctgctgaacgtgatccacacacctgatgccgtgacaagcctgtgcttcggcagatacggcagagaggacaacaccctgatcatgacaacaagaggcggcggactgatcatcaagatcctgaagagaaccgccgtgttcgtggaaggcggatctgaagttggacctcctccagctcaggccatgaagctgaatgtgcccagaaagacccggctgtacgtggaccagacactgagagaaagagaagccggcacagccatgcacagagccttccagactgacctgtacctgctgagactgagagccgccagagcctatctgcaggccctggaatctagcctgtctcctctgagcacaaccgccagagagcctctgaaactgcacgctgtggttcaaggcctgggacctaccttcaagctgaccctgcatctgcagaacaccagcaccacaagaccagtgctgggcctgctcgtgtgcttcctgtacaatgaggccctgtacagcctgccacgggccttttttaaggtgccactgctggtgcccggcctgaactaccctctggaaacctttgtggaaagcctgagcaacaagggcatcagcgacatcatcaaagtgctggtgctgagagagggccagtctgctcctctgctcagcgcccatgtgaatatgcctggctctgaaggcctggcagccgcttaagcgccgtcgac

SEQ ID NO: 17 - DNA, 3038 bp, Artificial sequence
  Construct comprising EFS promoter and COSEQ2-BBS1 nucleotide sequence (referred to as EFS-COSEQ2-BBS1)
actagtgggcagatctcgatcgagttgggccccagagcttggctccggtgcccgtcagtgggcagagcgcacatcgcccacagtccccgagaagttgtggggaggggtcggcaattgaaccggtgcctagagaaggtggcgcggggtaaactgggaaagtgatgtcgtgtactggctccgcctttttcccgagggtgggggagaaccgtatataagtgcagtagtcgccgtgaacgttctttttcgcaacgggtttgccgccagaacacaggtaagtgccgtgtgtggttcccgcgggcctggcctctttacgggttatggcccttgcgtgccttgaattacttccacctggctgcagtacgtgattcttgatcccgagcttcgggttggaagtgggtgggagagttcgaggccttgcgcttaaggagccccttcgcctcgtgcttgagttgaggcctggcctgggcgctggggccgccgcgtgcgaatctggtggcaccttcgcgcctgtctcgctgctttcgataagtctctagccatttaaaatttttgatgacctgctgcgacgctttttttctggcaagatagtcttgtaaatgcgggccaagatctgcacactggtatttcggtttttggggccgcgggcggcgacggggcccgtgcgtcccagcgcacatgttcggcgaggcggggcctgcgagcgcggccaccgagaatcggacgggggtagtctcaagctggccggcctgctctggtgcctggcctcgcgccgccgtgtatcgccccgccctgggcggcaaggctggcccggtcggcaccagttgcgtgagcggaaagatggccgcttcccggccctgctgcagggagctcaaaatggaggacgcggcgctcgggagagcgggcgggtgagtcacccacacaaaggaaaagggcctttccgtcctcagccgtcgcttcatgtgactccacggagtaccgggcgccgtccaggcacctcgattagttctcgagcttttggagtacgtcgtctttaggttggggggaggggttttatgcgatggagtttccccacactgagtgggtggagactgaagttaggccagcttggcacttgatgtaattctccttggaatttgccctttttgagtttggatcttggttcattctcaagcctcagacagtggttcaaagtttttttcttccatttcaggtgtcgtgaccatgagcttcgaattcgccaccatggctgccgcctctagctctgactctgatgcatgtggagcagagtctaacgaggccaatagcaagtggctggacgcccactacgatcctatggccaacatccacacattctctgcctgcctggccctggcagacctgcacggcgatggagagtataagctggtggtgggcgacctgggacctggcggccagcagccacggctgaaggtgctgaagggccctctggtcatgacagagtccccactgcccgccctgccagccgccgccgccaccttcctgatggagcagcacgagcctagaaccccagccctggccctggcctctggcccctgcgtgtacgtgtataagaacctgcggccctacttcaagtttagcctgccacagctgccccctaaccctctggagcaggatctgtggaatcaggccaaggaggacaggatcgatcctctgacactgaaggagatgctggagagcatccgggagacagccgaggagccactgagcatccagtccctgagattcctgcagctggagctgtccgagatggaggcctttgtgaaccagcacaagtctaatagcatcaagcgccagaccgtgatcaccacaatgaccacactgaagaagaacctggccgacgaggatgccgtgtcttgtctggtgctgggcacagagaataaggagctgctggtgctggacccagaggccttcaccatcctggccaagatgtctctgccctctgtgcccgtgttcctggaggtgagcggacagttcgacgtggagtttcggctggctgccgcctgcagaaacggcaatatctacatcctgcggagagatagcaagcacccaaagtattgtattgagctgtccgcccagcctgtgggcctgatcagagtgcacaaggtgctggtggtgggcagcacccaggactccctgcacggcttcacacacaagggcaagaagctgtggaccgtgcagatgcccgccgccatcctgaccatgaacctgctggagcagcacagcagaggcctgcaggccgtgatggcaggcctggcaaatggagaggtgaggatctaccgcgacaaggccctgctgaatgtgatccacacccctgatgccgtgacatccctgtgcttcggccggtatggcagagaggataacacactgatcatgaccacacggggcggcggcctgatcatcaagatcctgaagagaacagccgtgtttgtggagggcggctctgaagtgggcccaccccctgcccaggccatgaagctgaatgtgcccaggaagacccgcctgtacgtggaccagacactgagggaaagagaggcaggaacagcaatgcacagggccttccagaccgatctgtacctgctgagactgagagcagcaagagcctatctgcaggccctggagagctccctgtccccactgtctaccacagcaagagaacccctgaagctgcacgcagtggtgcagggcctgggacccaccttcaagctgacactgcacctgcagaacacatccaccacaaggcctgtgctgggcctgctggtgtgcttcctgtacaatgaggccctgtattctctgccacgcgccttctttaaggtgccactgctggtgcccggcctgaactatcccctggagacattcgtggagtccctgtctaataagggcatctctgatatcatcaaggtgctggtgctgagagaaggacagtccgcccctctgctgtctgcccacgtgaatatgccaggcagcgagggcctggctgccgcctgagcggccgcgtcgac

SEQ ID NO: 18 - DNA, 3073 bp, Artificial sequence
  Construct comprising UBC promoter and wild type BBS1 nucleotide sequence (referred to as UBC-WTBBS1)
actagtaacccgtgtcggctccagatctggcctccgcgccgggttttggcgcctcccgcgggcgcccccctcctcacggcgagcgctgccacgtcagacgaagggcgcagcgagcgtcctgatccttccgcccggacgctcaggacagcggcccgctgctcataagactcggccttagaaccccagtatcagcagaaggacattttaggacgggacttgggtgactctagggcactggttttctttccagagagcggaacaggcgaggaaaagtagtcccttctcggcgattctgcggagggatctccgtggggcggtgaacgccgatgattatataaggacgcgccgggtgtggcacagctagttccgtcgcagccgggatttgggtcgcggttcttgtttgtggatcgctgtgatcgtcacttggtgagtagcgggctgctgggctggccggggctttcgtggccgccgggccgctcggtgggacggaagcgtgtggagagaccgccaagggctgtagtctgggtccgcgagcaaggttgccctgaactgggggttggggggagcgcagcaaaatggcggctgttcccgagtcttgaatggaagacgcttgtgaggcgggctgtgaggtcgttgaaacaaggtggggggcatggtgggcggcaagaacccaaggtcttgaggccttcgctaatgcgggaaagctcttattcgggtgagatgggctggggcaccatctggggaccctgacgtgaagtttgtcactgactggagaactcggtttgtcgtctgttgcgggggcggcagttatggcggtgccgttgggcagtgcacccgtacctttgggagcgcgcgccctcgtcgtgtcgtgacgtcacccgttctgttggcttataatgcagggtggggccacctgccggtaggtgtgcggtaggcttttctccgtcgcaggacgcagggttcgggcctagggtaggctctcctgaatcgacaggcgccggacctctggtgaggggagggataagtgaggcgtcagtttctttggtcggttttatgtacctatcttcttaagtagctgaagctccggttttgaactatgcgctcggggttggcgagtgtgttttgtgaagttttttaggcaccttttgaaatgtaatcatttgggtcaatatgtaattttcagtgttagactagtaaattgtccgctaaattctggccgtttttggcttttttgttagacgaagcttgggctgcaggtcgagctcaagcttcgaattccgatggccgctgcgtcctcatcggattccgacgcctgcggagctgagagcaatgaggccaattcgaagtggttggatgcgcactacgacccaatggccaatatccacaccttttctgcctgcctagcgctggcagatttacatggggatggggaatacaagctggtggtaggggaccttggccctggtgggcagcagccccgcctgaaggtgctcaaaggaccactggtgatgaccgaaagcccgctacctgctctgccagctgctgctgccaccttcctcatggagcaacatgagccccggaccccagctctggcacttgcttcaggcccttgtgtctatgtgtataagaatctcagaccctacttcaagttcagcctgccccaattgcctccaaatcctctggaacaagacctttggaaccaggccaaagaggaccgaatcgaccccttaaccctgaaggagatgctggagagcatccgggagacggcagaggagcctttgtccatccagtcactcaggtttctgcagctggagctaagtgaaatggaggcatttgtaaaccaacacaagtccaactccatcaagcggcagacagtcatcaccaccatgaccaccttgaagaagaacctggctgacgaggatgctgtgtcttgcctggtgctgggcaccgagaacaaggagctcctggtgcttgaccccgaggccttcaccattttagccaagatgagccttcccagcgtccccgtcttcctagaggtttctggccagtttgatgttgagttccggcttgccgcggcctgccgcaatggaaacatctatattctgagaagagactccaagcaccccaagtactgcatcgagctgagcgcccagcctgtgggacttatccgggtacacaaggtcctagtggtgggcagcacccaagacagcctgcatggcttcacccacaaggggaagaagctgtggacagtgcagatgcccgcagccatcctgaccatgaacctcctggagcagcattcccggggcctgcaggccgtcatggctgggctggccaatggagaggtccgcatttatcgtgacaaggccctgctcaatgtcatccacaccccggatgcagtgaccagcctttgctttggccggtacgggcgggaggacaacaccctcatcatgaccactcgaggtggtggcctgatcatcaagatcctgaagcgtacagcagtgtttgtagagggaggaagtgaggtgggtcccccaccagcccaggccatgaaactcaatgtgccccgaaagacccggctttacgtggatcagacactgcgagagcgggaggctggcaccgccatgcaccgggccttccagacagacctatacctgctgcgcctacgtgctgcccgcgcctacctgcaggccctcgagtccagcctgagccccctgtccacgacagcccgagagccactcaagctgcacgccgtggttcagggccttggccccacctttaagctcacacttcacctgcagaacacctcaacaacccgtcctgtcctggggctgctggtctgcttcctgtacaacgaggcgctctattccctgccccgggccttcttcaaggtacccttgctggtgccagggctcaactaccccctggagacctttgtggagagtctcagtaacaagggcatctcagacatcatcaaggtgctggtgcttcgagaaggccaaagtgcacccctgctgagtgcccacgtcaacatgcctgggagcgaggggctggcggccgcctgagacttgtcgac

SEQ ID NO: 19 - DNA, 3080 bp, Artificial sequence
  Construct comprising UBC promoter and COSEQ1-BBS1 nucleotide sequence (referred to as UBC-COSEQ11BBS1)
actagtaacccgtgtcggctccagatctggcctccgcgccgggttttggcgcctcccgcgggcgcccccctcctcacggcgagcgctgccacgtcagacgaagggcgcagcgagcgtcctgatccttccgcccggacgctcaggacagcggcccgctgctcataagactcggccttagaaccccagtatcagcagaaggacattttaggacgggacttgggtgactctagggcactggttttctttccagagagcggaacaggcgaggaaaagtagtcccttctcggcgattctgcggagggatctccgtggggcggtgaacgccgatgattatataaggacgcgccgggtgtggcacagctagttccgtcgcagccgggatttgggtcgcggttcttgtttgtggatcgctgtgatcgtcacttggtgagtagcgggctgctgggctggccggggctttcgtggccgccgggccgctcggtgggacggaagcgtgtggagagaccgccaagggctgtagtctgggtccgcgagcaaggttgccctgaactgggggttggggggagcgcagcaaaatggcggctgttcccgagtcttgaatggaagacgcttgtgaggcgggctgtgaggtcgttgaaacaaggtggggggcatggtgggcggcaagaacccaaggtcttgaggccttcgctaatgcgggaaagctcttattcgggtgagatgggctggggcaccatctggggaccctgacgtgaagtttgtcactgactggagaactcggtttgtcgtctgttgcgggggcggcagttatggcggtgccgttgggcagtgcacccgtacctttgggagcgcgcgccctcgtcgtgtcgtgacgtcacccgttctgttggcttataatgcagggtggggccacctgccggtaggtgtgcggtaggcttttctccgtcgcaggacgcagggttcgggcctagggtaggctctcctgaatcgacaggcgccggacctctggtgaggggagggataagtgaggcgtcagtttctttggtcggttttatgtacctatcttcttaagtagctgaagctccggttttgaactatgcgctcggggttggcgagtgtgttttgtgaagttttttaggcaccttttgaaatgtaatcatttgggtcaatatgtaattttcagtgttagactagtaaattgtccgctaaattctggccgtttttggcttttttgttagacgaagcttgggctgcaggtcgagctcaagcttcgaattcgccaccatggctgccgccagcagttctgattctgatgcctgtggcgccgagagcaacgaggccaattctaaatggctggacgcccactacgaccccatggccaatatccacacctttagcgcctgtctggccctggctgatcttcatggcgacggcgagtataagctggttgtgggagatcttggacctggcggacagcagcctagactgaaggtgctgaagggccctctcgtgatgacagagtctcctcttcctgctctgcctgccgccgctgccacatttctgatggaacagcacgagcccagaacacccgctctggctcttgcttctggcccttgcgtgtacgtgtacaagaacctgcggccttacttcaagttcagcctgcctcagctgcctcctaatcctctggaacaggacctgtggaaccaggccaaagaggacagaatcgaccctctgacactgaaagagatgctggaatccatcagagagacagccgaggaacccctgtctatccagagcctgagattcctgcagctggaactgagcgagatggaagccttcgtgaaccagcacaagagcaacagcatcaagcggcagaccgtgatcaccaccatgaccacactgaagaagaacctggccgacgaggatgccgtgtcttgtctggtgctgggcaccgagaacaaagagctgctggttctggatcccgaggccttcacaatcctggccaagatgtctctgcctagcgtgcccgtgtttctggaagtgtccggccagttcgacgtggaatttcggctggccgctgcctgcagaaacggcaacatctacatcctgcggagggacagcaagcaccccaagtactgtatcgagctgtctgcccagcctgtgggcctgattagagtgcacaaggtgctggtcgtgggcagcacacaggatagcctgcacggctttacccacaagggcaagaaactgtggaccgtgcagatgccagccgccatcctgaccatgaatctgctcgaacagcacagcagaggactgcaggctgttatggcaggactggctaatggcgaagtgcggatctacagagacaaggccctgctgaacgtgatccacacacctgatgccgtgacaagcctgtgcttcggcagatacggcagagaggacaacaccctgatcatgacaacaagaggcggcggactgatcatcaagatcctgaagagaaccgccgtgttcgtggaaggcggatctgaagttggacctcctccagctcaggccatgaagctgaatgtgcccagaaagacccggctgtacgtggaccagacactgagagaaagagaagccggcacagccatgcacagagccttccagactgacctgtacctgctgagactgagagccgccagagcctatctgcaggccctggaatctagcctgtctcctctgagcacaaccgccagagagcctctgaaactgcacgctgtggttcaaggcctgggacctaccttcaagctgaccctgcatctgcagaacaccagcaccacaagaccagtgctgggcctgctcgtgtgcttcctgtacaatgaggccctgtacagcctgccacgggccttttttaaggtgccactgctggtgcccggcctgaactaccctctggaaacctttgtggaaagcctgagcaacaagggcatcagcgacatcatcaaagtgctggtgctgagagagggccagtctgctcctctgctcagcgcccatgtgaatatgcctggctctgaaggcctggcagccgcttaagcggccgcgtcgac

SEQ ID NO: 20 - DNA, 3080 bp, Artificial sequence
  Construct comprising UBC promoter and COSEQ2-BBS1 nucleotide sequence (referred to as UBC-COSEQ2-BBS1)
actagtaacccgtgtcggctccagatctggcctccgcgccgggttttggcgcctcccgcgggcgcccccctcctcacggcgagcgctgccacgtcagacgaagggcgcagcgagcgtcctgatccttccgcccggacgctcaggacagcggcccgctgctcataagactcggccttagaaccccagtatcagcagaaggacattttaggacgggacttgggtgactctagggcactggttttctttccagagagcggaacaggcgaggaaaagtagtcccttctcggcgattctgcggagggatctccgtggggcggtgaacgccgatgattatataaggacgcgccgggtgtggcacagctagttccgtcgcagccgggatttgggtcgcggttcttgtttgtggatcgctgtgatcgtcacttggtgagtagcgggctgctgggctggccggggctttcgtggccgccgggccgctcggtgggacggaagcgtgtggagagaccgccaagggctgtagtctgggtccgcgagcaaggttgccctgaactgggggttggggggagcgcagcaaaatggcggctgttcccgagtcttgaatggaagacgcttgtgaggcgggctgtgaggtcgttgaaacaaggtggggggcatggtgggcggcaagaacccaaggtcttgaggccttcgctaatgcgggaaagctcttattcgggtgagatgggctggggcaccatctggggaccctgacgtgaagtttgtcactgactggagaactcggtttgtcgtctgttgcgggggcggcagttatggcggtgccgttgggcagtgcacccgtacctttgggagcgcgcgccctcgtcgtgtcgtgacgtcacccgttctgttggcttataatgcagggtggggccacctgccggtaggtgtgcggtaggcttttctccgtcgcaggacgcagggttcgggcctagggtaggctctcctgaatcgacaggcgccggacctctggtgaggggagggataagtgaggcgtcagtttctttggtcggttttatgtacctatcttcttaagtagctgaagctccggttttgaactatgcgctcggggttggcgagtgtgttttgtgaagttttttaggcaccttttgaaatgtaatcatttgggtcaatatgtaattttcagtgttagactagtaaattgtccgctaaattctggccgtttttggcttttttgttagacgaagcttgggctgcaggtcgagctcaagcttcgaattcgccaccatggctgccgcctctagctctgactctgatgcatgtggagcagagtctaacgaggccaatagcaagtggctggacgcccactacgatcctatggccaacatccacacattctctgcctgcctggccctggcagacctgcacggcgatggagagtataagctggtggtgggcgacctgggacctggcggccagcagccacggctgaaggtgctgaagggccctctggtcatgacagagtccccactgcccgccctgccagccgccgccgccaccttcctgatggagcagcacgagcctagaaccccagccctggccctggcctctggcccctgcgtgtacgtgtataagaacctgcggccctacttcaagtttagcctgccacagctgccccctaaccctctggagcaggatctgtggaatcaggccaaggaggacaggatcgatcctctgacactgaaggagatgctggagagcatccgggagacagccgaggagccactgagcatccagtccctgagattcctgcagctggagctgtccgagatggaggcctttgtgaaccagcacaagtctaatagcatcaagcgccagaccgtgatcaccacaatgaccacactgaagaagaacctggccgacgaggatgccgtgtcttgtctggtgctgggcacagagaataaggagctgctggtgctggacccagaggccttcaccatcctggccaagatgtctctgccctctgtgcccgtgttcctggaggtgagcggacagttcgacgtggagtttcggctggctgccgcctgcagaaacggcaatatctacatcctgcggagagatagcaagcacccaaagtattgtattgagctgtccgcccagcctgtgggcctgatcagagtgcacaaggtgctggtggtgggcagcacccaggactccctgcacggcttcacacacaagggcaagaagctgtggaccgtgcagatgcccgccgccatcctgaccatgaacctgctggagcagcacagcagaggcctgcaggccgtgatggcaggcctggcaaatggagaggtgaggatctaccgcgacaaggccctgctgaatgtgatccacacccctgatgccgtgacatccctgtgcttcggccggtatggcagagaggataacacactgatcatgaccacacggggcggcggcctgatcatcaagatcctgaagagaacagccgtgtttgtggagggcggctctgaagtgggcccaccccctgcccaggccatgaagctgaatgtgcccaggaagacccgcctgtacgtggaccagacactgagggaaagagaggcaggaacagcaatgcacagggccttccagaccgatctgtacctgctgagactgagagcagcaagagcctatctgcaggccctggagagctccctgtccccactgtctaccacagcaagagaacccctgaagctgcacgcagtggtgcagggcctgggacccaccttcaagctgacactgcacctgcagaacacatccaccacaaggcctgtgctgggcctgctggtgtgcttcctgtacaatgaggccctgtattctctgccacgcgccttctttaaggtgccactgctggtgcccggcctgaactatcccctggagacattcgtggagtccctgtctaataagggcatctctgatatcatcaaggtgctggtgctgagagaaggacagtccgcccctctgctgtctgcccacgtgaatatgccaggcagcgagggcctggctgccgcctgagcggccgcgtcgac

SEQ ID NO: 21 - DNA, 2418 bp, Artificial sequence
  Construct comprising CMV promoter and wild type BBS1 nucleotide sequence (referred to as CMV-WTBBS1)
actagttattaatagtaatcaattacggggtcattagttcatagcccatatatggagttccgcgttacataacttacggtaaatggcccgcctggctgaccgcccaacgacccccgcccattgacgtcaataatgacgtatgttcccatagtaacgccaatagggactttccattgacgtcaatgggtggagtatttacggtaaactgcccacttggcagtacatcaagtgtatcatatgccaagtacgccccctattgacgtcaatgacggtaaatggcccgcctggcattatgcccagtacatgaccttatgggactttcctacttggcagtacatctacgtattagtcatcgctattaccatggtgatgcggttttggcagtacatcaatgggcgtggatagcggtttgactcacggggatttccaagtctccaccccattgacgtcaatgggagtttgttttggcaccaaaatcaacgggactttccaaaatgtcgtaacaactccgccccattgacgcaaatgggcggtaggcgtgtacggtgggaggtctatataagcagagctggtttagtgaaccgtcagatccgctagcgctaccggactcagatctcgaattccgatggccgctgcgtcctcatcggattccgacgcctgcggagctgagagcaatgaggccaattcgaagtggttggatgcgcactacgacccaatggccaatatccacaccttttctgcctgcctagcgctggcagatttacatggggatggggaatacaagctggtggtaggggaccttggccctggtgggcagcagccccgcctgaaggtgctcaaaggaccactggtgatgaccgaaagcccgctacctgctctgccagctgctgctgccaccttcctcatggagcaacatgagccccggaccccagctctggcacttgcttcaggcccttgtgtctatgtgtataagaatctcagaccctacttcaagttcagcctgccccaattgcctccaaatcctctggaacaagacctttggaaccaggccaaagaggaccgaatcgaccccttaaccctgaaggagatgctggagagcatccgggagacggcagaggagcctttgtccatccagtcactcaggtttctgcagctggagctaagtgaaatggaggcatttgtaaaccaacacaagtccaactccatcaagcggcagacagtcatcaccaccatgaccaccttgaagaagaacctggctgacgaggatgctgtgtcttgcctggtgctgggcaccgagaacaaggagctcctggtgcttgaccccgaggccttcaccattttagccaagatgagccttcccagcgtccccgtcttcctagaggtttctggccagtttgatgttgagttccggcttgccgcggcctgccgcaatggaaacatctatattctgagaagagactccaagcaccccaagtactgcatcgagctgagcgcccagcctgtgggacttatccgggtacacaaggtcctagtggtgggcagcacccaagacagcctgcatggcttcacccacaaggggaagaagctgtggacagtgcagatgcccgcagccatcctgaccatgaacctcctggagcagcattcccggggcctgcaggccgtcatggctgggctggccaatggagaggtccgcatttatcgtgacaaggccctgctcaatgtcatccacaccccggatgcagtgaccagcctttgctttggccggtacgggcgggaggacaacaccctcatcatgaccactcgaggtggtggcctgatcatcaagatcctgaagcgtacagcagtgtttgtagagggaggaagtgaggtgggtcccccaccagcccaggccatgaaactcaatgtgccccgaaagacccggctttacgtggatcagacactgcgagagcgggaggctggcaccgccatgcaccgggccttccagacagacctatacctgctgcgcctacgtgctgcccgcgcctacctgcaggccctcgagtccagcctgagccccctgtccacgacagcccgagagccactcaagctgcacgccgtggttcagggccttggccccacctttaagctcacacttcacctgcagaacacctcaacaacccgtcctgtcctggggctgctggtctgcttcctgtacaacgaggcgctctattccctgccccgggccttcttcaaggtacccttgctggtgccagggctcaactaccccctggagacctttgtggagagtctcagtaacaagggcatctcagacatcatcaaggtgctggtgcttcgagaaggccaaagtgcacccctgctgagtgcccacgtcaacatgcctgggagcgaggggctggcggccgcctgagacttgtcgac

SEQ ID NO: 22 - DNA, 2422 bp, Artificial sequence
  Construct comprising CMV promoter and COSEQ1-BBS1 nucleotide sequence (referred to as CMV-COSEQ1-BBS1)
actagttattaatagtaatcaattacggggtcattagttcatagcccatatatggagttccgcgttacataacttacggtaaatggcccgcctggctgaccgcccaacgacccccgcccattgacgtcaataatgacgtatgttcccatagtaacgccaatagggactttccattgacgtcaatgggtggagtatttacggtaaactgcccacttggcagtacatcaagtgtatcatatgccaagtacgccccctattgacgtcaatgacggtaaatggcccgcctggcattatgcccagtacatgaccttatgggactttcctacttggcagtacatctacgtattagtcatcgctattaccatggtgatgcggttttggcagtacatcaatgggcgtggatagcggtttgactcacggggatttccaagtctccaccccattgacgtcaatgggagtttgttttggcaccaaaatcaacgggactttccaaaatgtcgtaacaactccgccccattgacgcaaatgggcggtaggcgtgtacggtgggaggtctatataagcagagctggtttagtgaaccgtcagatccgctagcgctaccggactcagatctcgaattcgccaccatggctgccgccagcagttctgattctgatgcctgtggcgccgagagcaacgaggccaattctaaatggctggacgcccactacgaccccatggccaatatccacacctttagcgcctgtctggccctggctgatcttcatggcgacggcgagtataagctggttgtgggagatcttggacctggcggacagcagcctagactgaaggtgctgaagggccctctcgtgatgacagagtctcctcttcctgctctgcctgccgccgctgccacatttctgatggaacagcacgagcccagaacacccgctctggctcttgcttctggcccttgcgtgtacgtgtacaagaacctgcggccttacttcaagttcagcctgcctcagctgcctcctaatcctctggaacaggacctgtggaaccaggccaaagaggacagaatcgaccctctgacactgaaagagatgctggaatccatcagagagacagccgaggaacccctgtctatccagagcctgagattcctgcagctggaactgagcgagatggaagccttcgtgaaccagcacaagagcaacagcatcaagcggcagaccgtgatcaccaccatgaccacactgaagaagaacctggccgacgaggatgccgtgtcttgtctggtgctgggcaccgagaacaaagagctgctggttctggatcccgaggccttcacaatcctggccaagatgtctctgcctagcgtgcccgtgtttctggaagtgtccggccagttcgacgtggaatttcggctggccgctgcctgcagaaacggcaacatctacatcctgcggagggacagcaagcaccccaagtactgtatcgagctgtctgcccagcctgtgggcctgattagagtgcacaaggtgctggtcgtgggcagcacacaggatagcctgcacggctttacccacaagggcaagaaactgtggaccgtgcagatgccagccgccatcctgaccatgaatctgctcgaacagcacagcagaggactgcaggctgttatggcaggactggctaatggcgaagtgcggatctacagagacaaggccctgctgaacgtgatccacacacctgatgccgtgacaagcctgtgcttcggcagatacggcagagaggacaacaccctgatcatgacaacaagaggcggcggactgatcatcaagatcctgaagagaaccgccgtgttcgtggaaggcggatctgaagttggacctcctccagctcaggccatgaagctgaatgtgcccagaaagacccggctgtacgtggaccagacactgagagaaagagaagccggcacagccatgcacagagccttccagactgacctgtacctgctgagactgagagccgccagagcctatctgcaggccctggaatctagcctgtctcctctgagcacaaccgccagagagcctctgaaactgcacgctgtggttcaaggcctgggacctaccttcaagctgaccctgcatctgcagaacaccagcaccacaagaccagtgctgggcctgctcgtgtgcttcctgtacaatgaggccctgtacagcctgccacgggccttttttaaggtgccactgctggtgcccggcctgaactaccctctggaaacctttgtggaaagcctgagcaacaagggcatcagcgacatcatcaaagtgctggtgctgagagagggccagtctgctcctctgctcagcgcccatgtgaatatgcctggctctgaaggcctggcagccgcttaagcgccgtcgac

SEQ ID NO: 23 - DNA, 2425 bp, Artificial sequence
  Construct comprising CMV promoter and COSEQ2-BBS1 nucleotide sequence (referred to as CMV-COSEQ2-BBS1)
actagttattaatagtaatcaattacggggtcattagttcatagcccatatatggagttccgcgttacataacttacggtaaatggcccgcctggctgaccgcccaacgacccccgcccattgacgtcaataatgacgtatgttcccatagtaacgccaatagggactttccattgacgtcaatgggtggagtatttacggtaaactgcccacttggcagtacatcaagtgtatcatatgccaagtacgccccctattgacgtcaatgacggtaaatggcccgcctggcattatgcccagtacatgaccttatgggactttcctacttggcagtacatctacgtattagtcatcgctattaccatggtgatgcggttttggcagtacatcaatgggcgtggatagcggtttgactcacggggatttccaagtctccaccccattgacgtcaatgggagtttgttttggcaccaaaatcaacgggactttccaaaatgtcgtaacaactccgccccattgacgcaaatgggcggtaggcgtgtacggtgggaggtctatataagcagagctggtttagtgaaccgtcagatccgctagcgctaccggactcagatctcgaattcgccaccatggctgccgcctctagctctgactctgatgcatgtggagcagagtctaacgaggccaatagcaagtggctggacgcccactacgatcctatggccaacatccacacattctctgcctgcctggccctggcagacctgcacggcgatggagagtataagctggtggtgggcgacctgggacctggcggccagcagccacggctgaaggtgctgaagggccctctggtcatgacagagtccccactgcccgccctgccagccgccgccgccaccttcctgatggagcagcacgagcctagaaccccagccctggccctggcctctggcccctgcgtgtacgtgtataagaacctgcggccctacttcaagtttagcctgccacagctgccccctaaccctctggagcaggatctgtggaatcaggccaaggaggacaggatcgatcctctgacactgaaggagatgctggagagcatccgggagacagccgaggagccactgagcatccagtccctgagattcctgcagctggagctgtccgagatggaggcctttgtgaaccagcacaagtctaatagcatcaagcgccagaccgtgatcaccacaatgaccacactgaagaagaacctggccgacgaggatgccgtgtcttgtctggtgctgggcacagagaataaggagctgctggtgctggacccagaggccttcaccatcctggccaagatgtctctgccctctgtgcccgtgttcctggaggtgagcggacagttcgacgtggagtttcggctggctgccgcctgcagaaacggcaatatctacatcctgcggagagatagcaagcacccaaagtattgtattgagctgtccgcccagcctgtgggcctgatcagagtgcacaaggtgctggtggtgggcagcacccaggactccctgcacggcttcacacacaagggcaagaagctgtggaccgtgcagatgcccgccgccatcctgaccatgaacctgctggagcagcacagcagaggcctgcaggccgtgatggcaggcctggcaaatggagaggtgaggatctaccgcgacaaggccctgctgaatgtgatccacacccctgatgccgtgacatccctgtgcttcggccggtatggcagagaggataacacactgatcatgaccacacggggcggcggcctgatcatcaagatcctgaagagaacagccgtgtttgtggagggcggctctgaagtgggcccaccccctgcccaggccatgaagctgaatgtgcccaggaagacccgcctgtacgtggaccagacactgagggaaagagaggcaggaacagcaatgcacagggccttccagaccgatctgtacctgctgagactgagagcagcaagagcctatctgcaggccctggagagctccctgtccccactgtctaccacagcaagagaacccctgaagctgcacgcagtggtgcagggcctgggacccaccttcaagctgacactgcacctgcagaacacatccaccacaaggcctgtgctgggcctgctggtgtgcttcctgtacaatgaggccctgtattctctgccacgcgccttctttaaggtgccactgctggtgcccggcctgaactatcccctggagacattcgtggagtccctgtctaataagggcatctctgatatcatcaaggtgctggtgctgagagaaggacagtccgcccctctgctgtctgcccacgtgaatatgccaggcagcgagggcctggctgccgcctgagcggccgcgtcgac

SEQ ID NO: 24 - DNA, 2261 bp, Artificial sequence
  Construct comprising CBA promoter and wild type BBS1 nucleotide sequence (referred to as CBA-WTBBS1)
actagtgtacatctacgtattagtcatcgctattaccatggtcgaggtgagccccacgttctgcttcactctccccatctcccccccctccccacccccaattttgtatttatttattttttaattattttgtgcagcgatgggggcggggggggggggggggcgcgcgccaggcggggcggggcggggcgaggggcggggcggggcgaggcggagaggtgcggcggcagccaatcagagcggcgcgctccgaaagtttccttttatggcgaggcggcggcggcggcggccctataaaaagcgaagcgcgcggcgggcgggagtcgctgcgcgctgccttcgccccgtgccccgctccgccgccgcctcgcgccgcccgccccggctctgactgaccgcgttactcccacaggtgagcgggcgggacggcccttctcctccgggctgtaattagcgcttggaattccgatggccgctgcgtcctcatcggattccgacgcctgcggagctgagagcaatgaggccaattcgaagtggttggatgcgcactacgacccaatggccaatatccacaccttttctgcctgcctagcgctggcagatttacatggggatggggaatacaagctggtggtaggggaccttggccctggtgggcagcagccccgcctgaaggtgctcaaaggaccactggtgatgaccgaaagcccgctacctgctctgccagctgctgctgccaccttcctcatggagcaacatgagccccggaccccagctctggcacttgcttcaggcccttgtgtctatgtgtataagaatctcagaccctacttcaagttcagcctgccccaattgcctccaaatcctctggaacaagacctttggaaccaggccaaagaggaccgaatcgaccccttaaccctgaaggagatgctggagagcatccgggagacggcagaggagcctttgtccatccagtcactcaggtttctgcagctggagctaagtgaaatggaggcatttgtaaaccaacacaagtccaactccatcaagcggcagacagtcatcaccaccatgaccaccttgaagaagaacctggctgacgaggatgctgtgtcttgcctggtgctgggcaccgagaacaaggagctcctggtgcttgaccccgaggccttcaccattttagccaagatgagccttcccagcgtccccgtcttcctagaggtttctggccagtttgatgttgagttccggcttgccgcggcctgccgcaatggaaacatctatattctgagaagagactccaagcaccccaagtactgcatcgagctgagcgcccagcctgtgggacttatccgggtacacaaggtcctagtggtgggcagcacccaagacagcctgcatggcttcacccacaaggggaagaagctgtggacagtgcagatgcccgcagccatcctgaccatgaacctcctggagcagcattcccggggcctgcaggccgtcatggctgggctggccaatggagaggtccgcatttatcgtgacaaggccctgctcaatgtcatccacaccccggatgcagtgaccagcctttgctttggccggtacgggcgggaggacaacaccctcatcatgaccactcgaggtggtggcctgatcatcaagatcctgaagcgtacagcagtgtttgtagagggaggaagtgaggtgggtcccccaccagcccaggccatgaaactcaatgtgccccgaaagacccggctttacgtggatcagacactgcgagagcgggaggctggcaccgccatgcaccgggccttccagacagacctatacctgctgcgcctacgtgctgcccgcgcctacctgcaggccctcgagtccagcctgagccccctgtccacgacagcccgagagccactcaagctgcacgccgtggttcagggccttggccccacctttaagctcacacttcacctgcagaacacctcaacaacccgtcctgtcctggggctgctggtctgcttcctgtacaacgaggcgctctattccctgccccgggccttcttcaaggtacccttgctggtgccagggctcaactaccccctggagacctttgtggagagtctcagtaacaagggcatctcagacatcatcaaggtgctggtgcttcgagaaggccaaagtgcacccctgctgagtgcccacgtcaacatgcctgggagcgaggggctggcggccgcctgagacttgtcgac

SEQ ID NO: 25 - DNA, 2265 bp, Artificial sequence
  Construct comprising CBA promoter and COSEQ1-BBS1 nucleotide sequence (referred to as CBA-COSEQ1-BBS1)
actagtgtacatctacgtattagtcatcgctattaccatggtcgaggtgagccccacgttctgcttcactctccccatctcccccccctccccacccccaattttgtatttatttattttttaattattttgtgcagcgatgggggcggggggggggggggggcgcgcgccaggcggggcggggcggggcgaggggcggggcggggcgaggcggagaggtgcggcggcagccaatcagagcggcgcgctccgaaagtttccttttatggcgaggcggcggcggcggcggccctataaaaagcgaagcgcgcggcgggcgggagtcgctgcgcgctgccttcgccccgtgccccgctccgccgccgcctcgcgccgcccgccccggctctgactgaccgcgttactcccacaggtgagcgggcgggacggcccttctcctccgggctgtaattagcgcttggaattcgccaccatggctgccgccagcagttctgattctgatgcctgtggcgccgagagcaacgaggccaattctaaatggctggacgcccactacgaccccatggccaatatccacacctttagcgcctgtctggccctggctgatcttcatggcgacggcgagtataagctggttgtgggagatcttggacctggcggacagcagcctagactgaaggtgctgaagggccctctcgtgatgacagagtctcctcttcctgctctgcctgccgccgctgccacatttctgatggaacagcacgagcccagaacacccgctctggctcttgcttctggcccttgcgtgtacgtgtacaagaacctgcggccttacttcaagttcagcctgcctcagctgcctcctaatcctctggaacaggacctgtggaaccaggccaaagaggacagaatcgaccctctgacactgaaagagatgctggaatccatcagagagacagccgaggaacccctgtctatccagagcctgagattcctgcagctggaactgagcgagatggaagccttcgtgaaccagcacaagagcaacagcatcaagcggcagaccgtgatcaccaccatgaccacactgaagaagaacctggccgacgaggatgccgtgtcttgtctggtgctgggcaccgagaacaaagagctgctggttctggatcccgaggccttcacaatcctggccaagatgtctctgcctagcgtgcccgtgtttctggaagtgtccggccagttcgacgtggaatttcggctggccgctgcctgcagaaacggcaacatctacatcctgcggagggacagcaagcaccccaagtactgtatcgagctgtctgcccagcctgtgggcctgattagagtgcacaaggtgctggtcgtgggcagcacacaggatagcctgcacggctttacccacaagggcaagaaactgtggaccgtgcagatgccagccgccatcctgaccatgaatctgctcgaacagcacagcagaggactgcaggctgttatggcaggactggctaatggcgaagtgcggatctacagagacaaggccctgctgaacgtgatccacacacctgatgccgtgacaagcctgtgcttcggcagatacggcagagaggacaacaccctgatcatgacaacaagaggcggcggactgatcatcaagatcctgaagagaaccgccgtgttcgtggaaggcggatctgaagttggacctcctccagctcaggccatgaagctgaatgtgcccagaaagacccggctgtacgtggaccagacactgagagaaagagaagccggcacagccatgcacagagccttccagactgacctgtacctgctgagactgagagccgccagagcctatctgcaggccctggaatctagcctgtctcctctgagcacaaccgccagagagcctctgaaactgcacgctgtggttcaaggcctgggacctaccttcaagctgaccctgcatctgcagaacaccagcaccacaagaccagtgctgggcctgctcgtgtgcttcctgtacaatgaggccctgtacagcctgccacgggccttttttaaggtgccactgctggtgcccggcctgaactaccctctggaaacctttgtggaaagcctgagcaacaagggcatcagcgacatcatcaaagtgctggtgctgagagagggccagtctgctcctctgctcagcgcccatgtgaatatgcctggctctgaaggcctggcagccgcttaagcgccgtcgac

SEQ ID NO: 26 - DNA, 2268 bp, Artificial sequence
  Construct comprising CBA promoter and COSEQ2-BBS1 nucleotide sequence (referred to as CBA-COSEQ2-BBS1)
actagtgtacatctacgtattagtcatcgctattaccatggtcgaggtgagccccacgttctgcttcactctccccatctcccccccctccccacccccaattttgtatttatttattttttaattattttgtgcagcgatgggggcggggggggggggggggcgcgcgccaggcggggcggggcggggcgaggggcggggcggggcgaggcggagaggtgcggcggcagccaatcagagcggcgcgctccgaaagtttccttttatggcgaggcggcggcggcggcggccctataaaaagcgaagcgcgcggcgggcgggagtcgctgcgcgctgccttcgccccgtgccccgctccgccgccgcctcgcgccgcccgccccggctctgactgaccgcgttactcccacaggtgagcgggcgggacggcccttctcctccgggctgtaattagcgcttggaattcgccaccatggctgccgcctctagctctgactctgatgcatgtggagcagagtctaacgaggccaatagcaagtggctggacgcccactacgatcctatggccaacatccacacattctctgcctgcctggccctggcagacctgcacggcgatggagagtataagctggtggtgggcgacctgggacctggcggccagcagccacggctgaaggtgctgaagggccctctggtcatgacagagtccccactgcccgccctgccagccgccgccgccaccttcctgatggagcagcacgagcctagaaccccagccctggccctggcctctggcccctgcgtgtacgtgtataagaacctgcggccctacttcaagtttagcctgccacagctgccccctaaccctctggagcaggatctgtggaatcaggccaaggaggacaggatcgatcctctgacactgaaggagatgctggagagcatccgggagacagccgaggagccactgagcatccagtccctgagattcctgcagctggagctgtccgagatggaggcctttgtgaaccagcacaagtctaatagcatcaagcgccagaccgtgatcaccacaatgaccacactgaagaagaacctggccgacgaggatgccgtgtcttgtctggtgctgggcacagagaataaggagctgctggtgctggacccagaggccttcaccatcctggccaagatgtctctgccctctgtgcccgtgttcctggaggtgagcggacagttcgacgtggagtttcggctggctgccgcctgcagaaacggcaatatctacatcctgcggagagatagcaagcacccaaagtattgtattgagctgtccgcccagcctgtgggcctgatcagagtgcacaaggtgctggtggtgggcagcacccaggactccctgcacggcttcacacacaagggcaagaagctgtggaccgtgcagatgcccgccgccatcctgaccatgaacctgctggagcagcacagcagaggcctgcaggccgtgatggcaggcctggcaaatggagaggtgaggatctaccgcgacaaggccctgctgaatgtgatccacacccctgatgccgtgacatccctgtgcttcggccggtatggcagagaggataacacactgatcatgaccacacggggcggcggcctgatcatcaagatcctgaagagaacagccgtgtttgtggagggcggctctgaagtgggcccaccccctgcccaggccatgaagctgaatgtgcccaggaagacccgcctgtacgtggaccagacactgagggaaagagaggcaggaacagcaatgcacagggccttccagaccgatctgtacctgctgagactgagagcagcaagagcctatctgcaggccctggagagctccctgtccccactgtctaccacagcaagagaacccctgaagctgcacgcagtggtgcagggcctgggacccaccttcaagctgacactgcacctgcagaacacatccaccacaaggcctgtgctgggcctgctggtgtgcttcctgtacaatgaggccctgtattctctgccacgcgccttctttaaggtgccactgctggtgcccggcctgaactatcccctggagacattcgtggagtccctgtctaataagggcatctctgatatcatcaaggtgctggtgctgagagaaggacagtccgcccctctgctgtctgcccacgtgaatatgccaggcagcgagggcctggctgccgcctgagcggccgcgtcgac

SEQ ID NO: 27 - DNA, 2504 bp, Artificial sequence
  Construct comprising CAG promoter and wild type BBS1 nucleotide sequence (referred to as CAG-WTBBS1)
actagttcctggaggggtggagtcgtgacctaggccattgacgtcaataatgacgtatgttcccatagtaacgccaatagggactttccattgacgtcaatgggtggagtatttacggtaaactgcccacttggcagtacatcaagtgtatcatatgccaagtacgccccctattgacgtcaatgacggtaaatggcccgcctggcattatgcccagtacatgaccttatgggactttcctacttggcagtacatctacgtattagtcatcgctattaccatggtcgaggtgagccccacgttctgcttcactctccccatctcccccccctccccacccccaattttgtatttatttattttttaattattttgtgcagcgatgggggcggggggggggggggggcgcgcgccaggcggggcggggcggggcgaggggcggggcggggcgaggcggagaggtgcggcggcagccaatcagagcggcgcgctccgaaagtttccttttatggcgaggcggcggcggcggcggccctataaaaagcgaagcgcgcggcgggcgggagtcgctgcgcgctgccttcgccccgtgccccgctccgccgccgcctcgcgccgcccgccccggctctgactgaccgcgttactcccacaggtgagcgggcgggacggcccttctcctccgggctgtaattagcgcttggaattccgatggccgctgcgtcctcatcggattccgacgcctgcggagctgagagcaatgaggccaattcgaagtggttggatgcgcactacgacccaatggccaatatccacaccttttctgcctgcctagcgctggcagatttacatggggatggggaatacaagctggtggtaggggaccttggccctggtgggcagcagccccgcctgaaggtgctcaaaggaccactggtgatgaccgaaagcccgctacctgctctgccagctgctgctgccaccttcctcatggagcaacatgagccccggaccccagctctggcacttgcttcaggcccttgtgtctatgtgtataagaatctcagaccctacttcaagttcagcctgccccaattgcctccaaatcctctggaacaagacctttggaaccaggccaaagaggaccgaatcgaccccttaaccctgaaggagatgctggagagcatccgggagacggcagaggagcctttgtccatccagtcactcaggtttctgcagctggagctaagtgaaatggaggcatttgtaaaccaacacaagtccaactccatcaagcggcagacagtcatcaccaccatgaccaccttgaagaagaacctggctgacgaggatgctgtgtcttgcctggtgctgggcaccgagaacaaggagctcctggtgcttgaccccgaggccttcaccattttagccaagatgagccttcccagcgtccccgtcttcctagaggtttctggccagtttgatgttgagttccggcttgccgcggcctgccgcaatggaaacatctatattctgagaagagactccaagcaccccaagtactgcatcgagctgagcgcccagcctgtgggacttatccgggtacacaaggtcctagtggtgggcagcacccaagacagcctgcatggcttcacccacaaggggaagaagctgtggacagtgcagatgcccgcagccatcctgaccatgaacctcctggagcagcattcccggggcctgcaggccgtcatggctgggctggccaatggagaggtccgcatttatcgtgacaaggccctgctcaatgtcatccacaccccggatgcagtgaccagcctttgctttggccggtacgggcgggaggacaacaccctcatcatgaccactcgaggtggtggcctgatcatcaagatcctgaagcgtacagcagtgtttgtagagggaggaagtgaggtgggtcccccaccagcccaggccatgaaactcaatgtgccccgaaagacccggctttacgtggatcagacactgcgagagcgggaggctggcaccgccatgcaccgggccttccagacagacctatacctgctgcgcctacgtgctgcccgcgcctacctgcaggccctcgagtccagcctgagccccctgtccacgacagcccgagagccactcaagctgcacgccgtggttcagggccttggccccacctttaagctcacacttcacctgcagaacacctcaacaacccgtcctgtcctggggctgctggtctgcttcctgtacaacgaggcgctctattccctgccccgggccttcttcaaggtacccttgctggtgccagggctcaactaccccctggagacctttgtggagagtctcagtaacaagggcatctcagacatcatcaaggtgctggtgcttcgagaaggccaaagtgcacccctgctgagtgcccacgtcaacatgcctgggagcgaggggctggcggccgcctgagacttgtcgac

SEQ ID NO: 28 - DNA, 2508 bp, Artificial sequence
  Construct comprising CAG promoter and COSEQ1-BBS1 nucleotide sequence (referred to as CAG-COSEQ1-BBS1)
actagttcctggaggggtggagtcgtgacctaggccattgacgtcaataatgacgtatgttcccatagtaacgccaatagggactttccattgacgtcaatgggtggagtatttacggtaaactgcccacttggcagtacatcaagtgtatcatatgccaagtacgccccctattgacgtcaatgacggtaaatggcccgcctggcattatgcccagtacatgaccttatgggactttcctacttggcagtacatctacgtattagtcatcgctattaccatggtcgaggtgagccccacgttctgcttcactctccccatctcccccccctccccacccccaattttgtatttatttattttttaattattttgtgcagcgatgggggcggggggggggggggggcgcgcgccaggcggggcggggcggggcgaggggcggggcggggcgaggcggagaggtgcggcggcagccaatcagagcggcgcgctccgaaagtttccttttatggcgaggcggcggcggcggcggccctataaaaagcgaagcgcgcggcgggcgggagtcgctgcgcgctgccttcgccccgtgccccgctccgccgccgcctcgcgccgcccgccccggctctgactgaccgcgttactcccacaggtgagcgggcgggacggcccttctcctccgggctgtaattagcgcttggaattcgccaccatggctgccgccagcagttctgattctgatgcctgtggcgccgagagcaacgaggccaattctaaatggctggacgcccactacgaccccatggccaatatccacacctttagcgcctgtctggccctggctgatcttcatggcgacggcgagtataagctggttgtgggagatcttggacctggcggacagcagcctagactgaaggtgctgaagggccctctcgtgatgacagagtctcctcttcctgctctgcctgccgccgctgccacatttctgatggaacagcacgagcccagaacacccgctctggctcttgcttctggcccttgcgtgtacgtgtacaagaacctgcggccttacttcaagttcagcctgcctcagctgcctcctaatcctctggaacaggacctgtggaaccaggccaaagaggacagaatcgaccctctgacactgaaagagatgctggaatccatcagagagacagccgaggaacccctgtctatccagagcctgagattcctgcagctggaactgagcgagatggaagccttcgtgaaccagcacaagagcaacagcatcaagcggcagaccgtgatcaccaccatgaccacactgaagaagaacctggccgacgaggatgccgtgtcttgtctggtgctgggcaccgagaacaaagagctgctggttctggatcccgaggccttcacaatcctggccaagatgtctctgcctagcgtgcccgtgtttctggaagtgtccggccagttcgacgtggaatttcggctggccgctgcctgcagaaacggcaacatctacatcctgcggagggacagcaagcaccccaagtactgtatcgagctgtctgcccagcctgtgggcctgattagagtgcacaaggtgctggtcgtgggcagcacacaggatagcctgcacggctttacccacaagggcaagaaactgtggaccgtgcagatgccagccgccatcctgaccatgaatctgctcgaacagcacagcagaggactgcaggctgttatggcaggactggctaatggcgaagtgcggatctacagagacaaggccctgctgaacgtgatccacacacctgatgccgtgacaagcctgtgcttcggcagatacggcagagaggacaacaccctgatcatgacaacaagaggcggcggactgatcatcaagatcctgaagagaaccgccgtgttcgtggaaggcggatctgaagttggacctcctccagctcaggccatgaagctgaatgtgcccagaaagacccggctgtacgtggaccagacactgagagaaagagaagccggcacagccatgcacagagccttccagactgacctgtacctgctgagactgagagccgccagagcctatctgcaggccctggaatctagcctgtctcctctgagcacaaccgccagagagcctctgaaactgcacgctgtggttcaaggcctgggacctaccttcaagctgaccctgcatctgcagaacaccagcaccacaagaccagtgctgggcctgctcgtgtgcttcctgtacaatgaggccctgtacagcctgccacgggccttttttaaggtgccactgctggtgcccggcctgaactaccctctggaaacctttgtggaaagcctgagcaacaagggcatcagcgacatcatcaaagtgctggtgctgagagagggccagtctgctcctctgctcagcgcccatgtgaatatgcctggctctgaaggcctggcagccgcttaagcgccgtcgac

SEQ ID NO: 29 - DNA, 2511 bp, Artificial sequence
  Construct comprising CAG promoter and COSEQ2-BBS1 nucleotide sequence (referred to as CAG-COSEQ2-BBS1)
actagttcctggaggggtggagtcgtgacctaggccattgacgtcaataatgacgtatgttcccatagtaacgccaatagggactttccattgacgtcaatgggtggagtatttacggtaaactgcccacttggcagtacatcaagtgtatcatatgccaagtacgccccctattgacgtcaatgacggtaaatggcccgcctggcattatgcccagtacatgaccttatgggactttcctacttggcagtacatctacgtattagtcatcgctattaccatggtcgaggtgagccccacgttctgcttcactctccccatctcccccccctccccacccccaattttgtatttatttattttttaattattttgtgcagcgatgggggcggggggggggggggggcgcgcgccaggcggggcggggcggggcgaggggcggggcggggcgaggcggagaggtgcggcggcagccaatcagagcggcgcgctccgaaagtttccttttatggcgaggcggcggcggcggcggccctataaaaagcgaagcgcgcggcgggcgggagtcgctgcgcgctgccttcgccccgtgccccgctccgccgccgcctcgcgccgcccgccccggctctgactgaccgcgttactcccacaggtgagcgggcgggacggcccttctcctccgggctgtaattagcgcttggaattcgccaccatggctgccgcctctagctctgactctgatgcatgtggagcagagtctaacgaggccaatagcaagtggctggacgcccactacgatcctatggccaacatccacacattctctgcctgcctggccctggcagacctgcacggcgatggagagtataagctggtggtgggcgacctgggacctggcggccagcagccacggctgaaggtgctgaagggccctctggtcatgacagagtccccactgcccgccctgccagccgccgccgccaccttcctgatggagcagcacgagcctagaaccccagccctggccctggcctctggcccctgcgtgtacgtgtataagaacctgcggccctacttcaagtttagcctgccacagctgccccctaaccctctggagcaggatctgtggaatcaggccaaggaggacaggatcgatcctctgacactgaaggagatgctggagagcatccgggagacagccgaggagccactgagcatccagtccctgagattcctgcagctggagctgtccgagatggaggcctttgtgaaccagcacaagtctaatagcatcaagcgccagaccgtgatcaccacaatgaccacactgaagaagaacctggccgacgaggatgccgtgtcttgtctggtgctgggcacagagaataaggagctgctggtgctggacccagaggccttcaccatcctggccaagatgtctctgccctctgtgcccgtgttcctggaggtgagcggacagttcgacgtggagtttcggctggctgccgcctgcagaaacggcaatatctacatcctgcggagagatagcaagcacccaaagtattgtattgagctgtccgcccagcctgtgggcctgatcagagtgcacaaggtgctggtggtgggcagcacccaggactccctgcacggcttcacacacaagggcaagaagctgtggaccgtgcagatgcccgccgccatcctgaccatgaacctgctggagcagcacagcagaggcctgcaggccgtgatggcaggcctggcaaatggagaggtgaggatctaccgcgacaaggccctgctgaatgtgatccacacccctgatgccgtgacatccctgtgcttcggccggtatggcagagaggataacacactgatcatgaccacacggggcggcggcctgatcatcaagatcctgaagagaacagccgtgtttgtggagggcggctctgaagtgggcccaccccctgcccaggccatgaagctgaatgtgcccaggaagacccgcctgtacgtggaccagacactgagggaaagagaggcaggaacagcaatgcacagggccttccagaccgatctgtacctgctgagactgagagcagcaagagcctatctgcaggccctggagagctccctgtccccactgtctaccacagcaagagaacccctgaagctgcacgcagtggtgcagggcctgggacccaccttcaagctgacactgcacctgcagaacacatccaccacaaggcctgtgctgggcctgctggtgtgcttcctgtacaatgaggccctgtattctctgccacgcgccttctttaaggtgccactgctggtgcccggcctgaactatcccctggagacattcgtggagtccctgtctaataagggcatctctgatatcatcaaggtgctggtgctgagagaaggacagtccgcccctctgctgtctgcccacgtgaatatgccaggcagcgagggcctggctgccgcctgagcggccgcgtcgac

SEQ ID NO: 30 - DNA, 3428 bp, Artificial sequence
  Construct comprising EFS promoter and wild type BBS10 nucleotide sequence (referred to as EFS-WTBBS10)
actagtgggcagatctcgatcgagttgggccccagagcttggctccggtgcccgtcagtgggcagagcgcacatcgcccacagtccccgagaagttgtggggaggggtcggcaattgaaccggtgcctagagaaggtggcgcggggtaaactgggaaagtgatgtcgtgtactggctccgcctttttcccgagggtgggggagaaccgtatataagtgcagtagtcgccgtgaacgttctttttcgcaacgggtttgccgccagaacacaggtaagtgccgtgtgtggttcccgcgggcctggcctctttacgggttatggcccttgcgtgccttgaattacttccacctggctgcagtacgtgattcttgatcccgagcttcgggttggaagtgggtgggagagttcgaggccttgcgcttaaggagccccttcgcctcgtgcttgagttgaggcctggcctgggcgctggggccgccgcgtgcgaatctggtggcaccttcgcgcctgtctcgctgctttcgataagtctctagccatttaaaatttttgatgacctgctgcgacgctttttttctggcaagatagtcttgtaaatgcgggccaagatctgcacactggtatttcggtttttggggccgcgggcggcgacggggcccgtgcgtcccagcgcacatgttcggcgaggcggggcctgcgagcgcggccaccgagaatcggacgggggtagtctcaagctggccggcctgctctggtgcctggcctcgcgccgccgtgtatcgccccgccctgggcggcaaggctggcccggtcggcaccagttgcgtgagcggaaagatggccgcttcccggccctgctgcagggagctcaaaatggaggacgcggcgctcgggagagcgggcgggtgagtcacccacacaaaggaaaagggcctttccgtcctcagccgtcgcttcatgtgactccacggagtaccgggcgccgtccaggcacctcgattagttctcgagcttttggagtacgtcgtctttaggttggggggaggggttttatgcgatggagtttccccacactgagtgggtggagactgaagttaggccagcttggcacttgatgtaattctccttggaatttgccctttttgagtttggatcttggttcattctcaagcctcagacagtggttcaaagtttttttcttccatttcaggtgtcgtgaccatgagcttcgaattcgccaccatgttaagttctatggccgctgcagggtctgtgaaggcggcgttgcaggtggccgaggtgctggaagccatcgtgagctgctgcgtggggcccgagggacggcaagttttgtgtacgaagcccactggcgaggtgcttctcagccggaatggaggccgcctcctggaggcgctacacttagagcatcccatagccaggatgatagtggactgtgtttccagtcatctcaaaaaaacaggagatggtgcaaaaacatttattatctttctttgccatttgcttagaggacttcatgcaatcacagacagagaaaaggatcctttgatgtgtgaaaacattcaaacccatggaaggcattggaaaaattgttctcggtggaaatttatttcccaggctctcctaacgtttcagacacaaatattagacggtattatggaccagtacctaagtagacactttttgtctatcttttcgtctgctaaagagagaacattgtgtaggagctctttagagttgctcttagaagcatacttttgtggaagagtgggaagaaataatcataaatttatttcacagttgatgtgtgactactttttcaagtgtatgacttgtaaaagtgggattggtgtatttgagttagtggatgaccattttgtagagttgaatgttggtgtcactggccttcctgtttcagattccaggatcatagctggtcttgtgcttcagaaagatttttctgtgtaccgcccagcagatggtgacatgcgaatggtgatagtaacagaaaccattcagcctcttttttccacttctggatcagagtttattctaaattcagaagcacagtttcagacatctcaattttggattatggaaaagacaaaagcaataatgaaacatctacatagtcagaatgtaaaattgctcatatctagtgtgaaacaaccagatttagttagttattatgcaggggtgaatggcatatcagtggttgagtgtttatcatcagaagaagtttctcttatccggaggatcattggtctttctccatttgtaccaccacaggccttttcgcagtgtgaaatacctaacactgctttggtgaaattttgtaaacctcttatccttagatccaaaagatatgttcatctaggcttgataagcacatgtgcatttataccacactctatagttctttgtggaccagtgcatggtctcattgaacaacatgaggatgctttacatggagcacttaaaatgcttcggcaattatttaaagaccttgatctaaattacatgacacaaaccaatgaccaaaatggcacttcaagtctttttatttataagaacagtggagaaagttatcaagcaccagatcctggtaatggctcaatacaaaggccttatcaggacacagttgcagagaacaaagatgcattggaaaaaactcaaacatatttaaaagtacattctaatttggtaattccagatgtagaattagaaacatatattccgtattcaacccccacactgacaccaacagatacattccaaacagttgaaacgctgacatgtttgtctttggaaagaaacaggctaactgattattatgaaccattactcaagaacaattccactgcttattcaacaaggggaaatagaatagaaatttcttacgaaaatttacaggtcacaaatattactagaaagggaagcatgttaccagtgagctgtaagttaccgaatatgggtacttcccagagttacctttcctcatctatgccagctggttgtgttttgccagtaggtggtaattttgagatcttgttacattactatcttctcaattatgccaaaaaatgccatcaatcagaagaaaccatggttagtatgataatagctaatgcacttttaggcattcccaaagtcctttataaatctaaaacaggaaagtacagctttccacatacatatataagagctgtccatgcactgcaaaccaatcaacccttggtaagcagtcagacaggtttggaatcagtaatgggtaaataccagctactaacttcagttcttcagtgtttgacaaaaatattaaccattgacatggtaatcactgttaagagacaccctcagaaagttcacaatcaagattcagaagatgaactataagcggccgcgtcgac

SEQ ID NO: 31 - DNA, 3425 bp, Artificial sequence
  Construct comprising EFS promoter and COSEQ1-BBS10 nucleotide sequence (referred to as EFS-COSEQ1-BBS10)
actagtgggcagatctcgatcgagttgggccccagagcttggctccggtgcccgtcagtgggcagagcgcacatcgcccacagtccccgagaagttgtggggaggggtcggcaattgaaccggtgcctagagaaggtggcgcggggtaaactgggaaagtgatgtcgtgtactggctccgcctttttcccgagggtgggggagaaccgtatataagtgcagtagtcgccgtgaacgttctttttcgcaacgggtttgccgccagaacacaggtaagtgccgtgtgtggttcccgcgggcctggcctctttacgggttatggcccttgcgtgccttgaattacttccacctggctgcagtacgtgattcttgatcccgagcttcgggttggaagtgggtgggagagttcgaggccttgcgcttaaggagccccttcgcctcgtgcttgagttgaggcctggcctgggcgctggggccgccgcgtgcgaatctggtggcaccttcgcgcctgtctcgctgctttcgataagtctctagccatttaaaatttttgatgacctgctgcgacgctttttttctggcaagatagtcttgtaaatgcgggccaagatctgcacactggtatttcggtttttggggccgcgggcggcgacggggcccgtgcgtcccagcgcacatgttcggcgaggcggggcctgcgagcgcggccaccgagaatcggacgggggtagtctcaagctggccggcctgctctggtgcctggcctcgcgccgccgtgtatcgccccgccctgggcggcaaggctggcccggtcggcaccagttgcgtgagcggaaagatggccgcttcccggccctgctgcagggagctcaaaatggaggacgcggcgctcgggagagcgggcgggtgagtcacccacacaaaggaaaagggcctttccgtcctcagccgtcgcttcatgtgactccacggagtaccgggcgccgtccaggcacctcgattagttctcgagcttttggagtacgtcgtctttaggttggggggaggggttttatgcgatggagtttccccacactgagtgggtggagactgaagttaggccagcttggcacttgatgtaattctccttggaatttgccctttttgagtttggatcttggttcattctcaagcctcagacagtggttcaaagtttttttcttccatttcaggtgtcgtgaccatgagcttcgaattcgccaccatgctgtctagcatggctgccgctggatctgtgaaagctgctctgcaggttgccgaggtgctggaagccatcgtgtcttgttgtgtgggacctgagggcagacaggtgctgtgtacaaagcctacaggcgaagtgctgctgagcagaaatggcggcagactgctcgaagccctgcacctggaacaccctatcgccagaatgatcgtggactgcgtgtccagccacctgaagaaaacaggcgacggcgccaagaccttcatcatctttctgtgccatctgctgcggggcctgcacgccatcaccgatagagaaaaggaccctctgatgtgcgagaacatccagacacacggccggcactggaagaactgctcccggtggaagtttatcagccaggctctgctgacctttcagacccagatcctggacggcatcatggaccagtacctgagcagacacttcctgagcatcttcagcagcgccaaagaacggaccctgtgcagaagctctctggaactgctgctcgaggcctacttttgcggcagagtgggcagaaacaaccacaagttcatctcccagctgatgtgtgactacttcttcaagtgcatgacctgcaagagcggcatcggcgtgttcgagctggtggacgatcacttcgtggaactgaatgtgggcgtgaccggcctgcctgtgtccgatagcagaattattgccggcctggtgctgcagaaagacttcagcgtgtacagacccgccgacggcgacatgagaatggtcatcgtgaccgagacaatccagcctctgttcagcacaagcggcagcgagttcatcctgaacagcgaggcccagtttcagaccagccagttctggatcatggaaaagaccaaggccatcatgaagcacctccacagccagaacgtgaagctgctgatctccagcgtgaagcagcccgacctggtgtcttattatgccggcgtgaacggcatcagcgtggtggaatgtctgagcagcgaagaggtgtccctgatcagacggatcatcggactgagcccctttgtgcctcctcaagcctttagccagtgcgagatccctaacacagccctggtcaagttctgcaagcccctgatcctgcggagcaagagatatgtgcacctgggcctgatcagcacatgcgccttcattcctcactccatcgtgctgtgtggacctgtgcacggactgattgagcagcacgaagatgcactgcacggcgccctgaaaatgctgagacagctgttcaaggacctggacctgaactacatgacccagaccaacgaccagaacggcaccagcagcctgttcatctacaagaacagcggcgagagctatcaggccccagatccaggcaatggcagcatccagaggccttaccaggataccgtggccgagaacaaggacgccctggaaaaaacccagacctacctgaaggtgcacagcaacctggtcatccccgatgtggaactggaaacctacattccctacagcacccctacactgacccctaccgataccttccagaccgtggaaaccctgacctgtctgagcctggaacggaacagactgaccgactactacgagcccctgctgaaaaacaacagcaccgcctatagcacccggggcaacagaatcgagatcagctacgagaacctgcaagtgaccaacatcacccggaagggctccatgctgccagtgtcctgcaagctgcctaatatgggcaccagccagagctacctgtcctcttctatgcctgccggatgtgtgctgcctgtcggcggcaattttgagatcctgctgcactactacctgctgaactacgccaagaagtgccaccagagcgaagagacaatggtgtccatgattatcgccaacgctctgctgggcatccccaaggtgctgtacaagagcaagaccggcaagtacagcttccctcacacctacattagagccgtgcacgccctgcagaccaatcagccactggtttctagccagacaggcctggaaagcgtgatgggaaagtaccagctgctgaccagcgtgctgcagtgcctgaccaagatcctgaccatcgacatggtcatcaccgtgaagcggcaccctcagaaagtgcacaaccaggacagcgaggacgagctgtaggcgccgtcgac

SEQ ID NO: 32 - DNA, 3428 bp, Artificial sequence
  Construct comprising EFS promoter and COSEQ2-BBS10 nucleotide sequence (referred to as EFS-COSEQ2-BBS10)
actagtgggcagatctcgatcgagttgggccccagagcttggctccggtgcccgtcagtgggcagagcgcacatcgcccacagtccccgagaagttgtggggaggggtcggcaattgaaccggtgcctagagaaggtggcgcggggtaaactgggaaagtgatgtcgtgtactggctccgcctttttcccgagggtgggggagaaccgtatataagtgcagtagtcgccgtgaacgttctttttcgcaacgggtttgccgccagaacacaggtaagtgccgtgtgtggttcccgcgggcctggcctctttacgggttatggcccttgcgtgccttgaattacttccacctggctgcagtacgtgattcttgatcccgagcttcgggttggaagtgggtgggagagttcgaggccttgcgcttaaggagccccttcgcctcgtgcttgagttgaggcctggcctgggcgctggggccgccgcgtgcgaatctggtggcaccttcgcgcctgtctcgctgctttcgataagtctctagccatttaaaatttttgatgacctgctgcgacgctttttttctggcaagatagtcttgtaaatgcgggccaagatctgcacactggtatttcggtttttggggccgcgggcggcgacggggcccgtgcgtcccagcgcacatgttcggcgaggcggggcctgcgagcgcggccaccgagaatcggacgggggtagtctcaagctggccggcctgctctggtgcctggcctcgcgccgccgtgtatcgccccgccctgggcggcaaggctggcccggtcggcaccagttgcgtgagcggaaagatggccgcttcccggccctgctgcagggagctcaaaatggaggacgcggcgctcgggagagcgggcgggtgagtcacccacacaaaggaaaagggcctttccgtcctcagccgtcgcttcatgtgactccacggagtaccgggcgccgtccaggcacctcgattagttctcgagcttttggagtacgtcgtctttaggttggggggaggggttttatgcgatggagtttccccacactgagtgggtggagactgaagttaggccagcttggcacttgatgtaattctccttggaatttgccctttttgagtttggatcttggttcattctcaagcctcagacagtggttcaaagtttttttcttccatttcaggtgtcgtgaccatgagcttcgaattcgccaccatgctgagctccatggctgccgccggatctgtgaaagccgccctgcaggtggcagaggtgctggaggcaatcgtgagctgttgcgtgggacctgagggccggcaggtgctgtgcacaaagccaaccggcgaggtgctgctgtctagaaatggcggccggctgctggaggccctgcacctggagcacccaattgcaagaatgatcgtggactgcgtgtctagccacctgaagaagacaggcgatggcgccaagaccttcatcatcttcctgtgccacctgctgaggggcctgcacgccatcacagaccgcgagaaggatcctctgatgtgcgagaacatccagacccacggcaggcactggaagaattgttcccgctggaagttcatctctcaggccctgctgacatttcagacccagatcctggacggcatcatggatcagtatctgagcaggcacttcctgtccatcttttcctctgccaaggagcggaccctgtgcagaagctccctggagctgctgctggaggcctacttctgtggccgggtgggcagaaacaatcacaagtttatcagccagctgatgtgcgactatttctttaagtgcatgacctgtaagtccggcatcggcgtgttcgagctggtggacgatcactttgtggagctgaacgtgggagtgacaggcctgcccgtgtccgactctcgcatcatcgccggcctggtgctgcagaaggatttctccgtgtaccggcctgccgacggcgatatgagaatggtcatcgtgaccgagacaatccagccactgttcagcacctccggctctgagttcatcctgaacagcgaggcccagttccagacatctcagttttggatcatggagaagaccaaggccatcatgaagcacctgcacagccagaacgtgaagctgctgatctctagcgtgaagcagccagacctggtgtcttactatgccggcgtgaatggcatcagcgtggtggagtgtctgtcctctgaggaggtgtccctgatccggagaatcattggcctgtctcccttcgtgccccctcaggcctttagccagtgcgagatccccaacacagccctggtgaagttctgtaagcctctgatcctgaggtccaagcggtacgtgcacctgggcctgatcagcacctgcgcctttatcccacactctatcgtgctgtgcggacctgtgcacggcctgattgagcagcacgaggatgcactgcacggcgccctgaagatgctgaggcagctgttcaaggacctggatctgaattacatgacccagacaaacgaccagaatggcacaagctccctgtttatctacaagaactctggcgagagctatcaggccccagatcccggcaatggcagcattcagcgcccctaccaggacacagtggcagagaacaaggatgccctggagaagacccagacatatctgaaggtgcactccaacctggtcatccctgacgtggagctggagacatacatcccttattctaccccaacactgacccccacagataccttccagacagtggagacactgacctgcctgtccctggagaggaaccgcctgaccgactactatgagcccctgctgaagaacaattccacagcctactctacccggggcaatagaatcgagatcagctatgagaacctgcaggtgacaaatatcaccagaaagggctctatgctgcctgtgagctgcaagctgccaaacatgggcaccagccagtcctacctgtctagctccatgcctgcaggatgcgtgctgcctgtgggcggcaacttcgagatcctgctgcactactatctgctgaattatgccaagaagtgccaccagagcgaggagacaatggtgtccatgatcatcgccaacgccctgctgggcatcccaaaggtgctgtacaagtctaagaccggcaagtacagctttccccacacctatatccgggccgtgcacgccctgcagacaaatcagcctctggtgtctagccagaccggcctggagtccgtgatgggcaagtaccagctgctgacatctgtgctgcagtgtctgacaaagatcctgaccatcgatatggtcatcaccgtgaagagacacccacagaaggtgcacaatcaggacagcgaggatgagctgtaagcggccgcgtcgac

SEQ ID NO: 33 - DNA, 3470 bp, Artificial sequence
  Construct comprising UBC promoter and wild type BBS10 nucleotide sequence (referred to as UBC-WTBBS10)
actagtaacccgtgtcggctccagatctggcctccgcgccgggttttggcgcctcccgcgggcgcccccctcctcacggcgagcgctgccacgtcagacgaagggcgcagcgagcgtcctgatccttccgcccggacgctcaggacagcggcccgctgctcataagactcggccttagaaccccagtatcagcagaaggacattttaggacgggacttgggtgactctagggcactggttttctttccagagagcggaacaggcgaggaaaagtagtcccttctcggcgattctgcggagggatctccgtggggcggtgaacgccgatgattatataaggacgcgccgggtgtggcacagctagttccgtcgcagccgggatttgggtcgcggttcttgtttgtggatcgctgtgatcgtcacttggtgagtagcgggctgctgggctggccggggctttcgtggccgccgggccgctcggtgggacggaagcgtgtggagagaccgccaagggctgtagtctgggtccgcgagcaaggttgccctgaactgggggttggggggagcgcagcaaaatggcggctgttcccgagtcttgaatggaagacgcttgtgaggcgggctgtgaggtcgttgaaacaaggtggggggcatggtgggcggcaagaacccaaggtcttgaggccttcgctaatgcgggaaagctcttattcgggtgagatgggctggggcaccatctggggaccctgacgtgaagtttgtcactgactggagaactcggtttgtcgtctgttgcgggggcggcagttatggcggtgccgttgggcagtgcacccgtacctttgggagcgcgcgccctcgtcgtgtcgtgacgtcacccgttctgttggcttataatgcagggtggggccacctgccggtaggtgtgcggtaggcttttctccgtcgcaggacgcagggttcgggcctagggtaggctctcctgaatcgacaggcgccggacctctggtgaggggagggataagtgaggcgtcagtttctttggtcggttttatgtacctatcttcttaagtagctgaagctccggttttgaactatgcgctcggggttggcgagtgtgttttgtgaagttttttaggcaccttttgaaatgtaatcatttgggtcaatatgtaattttcagtgttagactagtaaattgtccgctaaattctggccgtttttggcttttttgttagacgaagcttgggctgcaggtcgagctcaagcttcgaattcgccaccatgttaagttctatggccgctgcagggtctgtgaaggcggcgttgcaggtggccgaggtgctggaagccatcgtgagctgctgcgtggggcccgagggacggcaagttttgtgtacgaagcccactggcgaggtgcttctcagccggaatggaggccgcctcctggaggcgctacacttagagcatcccatagccaggatgatagtggactgtgtttccagtcatctcaaaaaaacaggagatggtgcaaaaacatttattatctttctttgccatttgcttagaggacttcatgcaatcacagacagagaaaaggatcctttgatgtgtgaaaacattcaaacccatggaaggcattggaaaaattgttctcggtggaaatttatttcccaggctctcctaacgtttcagacacaaatattagacggtattatggaccagtacctaagtagacactttttgtctatcttttcgtctgctaaagagagaacattgtgtaggagctctttagagttgctcttagaagcatacttttgtggaagagtgggaagaaataatcataaatttatttcacagttgatgtgtgactactttttcaagtgtatgacttgtaaaagtgggattggtgtatttgagttagtggatgaccattttgtagagttgaatgttggtgtcactggccttcctgtttcagattccaggatcatagctggtcttgtgcttcagaaagatttttctgtgtaccgcccagcagatggtgacatgcgaatggtgatagtaacagaaaccattcagcctcttttttccacttctggatcagagtttattctaaattcagaagcacagtttcagacatctcaattttggattatggaaaagacaaaagcaataatgaaacatctacatagtcagaatgtaaaattgctcatatctagtgtgaaacaaccagatttagttagttattatgcaggggtgaatggcatatcagtggttgagtgtttatcatcagaagaagtttctcttatccggaggatcattggtctttctccatttgtaccaccacaggccttttcgcagtgtgaaatacctaacactgctttggtgaaattttgtaaacctcttatccttagatccaaaagatatgttcatctaggcttgataagcacatgtgcatttataccacactctatagttctttgtggaccagtgcatggtctcattgaacaacatgaggatgctttacatggagcacttaaaatgcttcggcaattatttaaagaccttgatctaaattacatgacacaaaccaatgaccaaaatggcacttcaagtctttttatttataagaacagtggagaaagttatcaagcaccagatcctggtaatggctcaatacaaaggccttatcaggacacagttgcagagaacaaagatgcattggaaaaaactcaaacatatttaaaagtacattctaatttggtaattccagatgtagaattagaaacatatattccgtattcaacccccacactgacaccaacagatacattccaaacagttgaaacgctgacatgtttgtctttggaaagaaacaggctaactgattattatgaaccattactcaagaacaattccactgcttattcaacaaggggaaatagaatagaaatttcttacgaaaatttacaggtcacaaatattactagaaagggaagcatgttaccagtgagctgtaagttaccgaatatgggtacttcccagagttacctttcctcatctatgccagctggttgtgttttgccagtaggtggtaattttgagatcttgttacattactatcttctcaattatgccaaaaaatgccatcaatcagaagaaaccatggttagtatgataatagctaatgcacttttaggcattcccaaagtcctttataaatctaaaacaggaaagtacagctttccacatacatatataagagctgtccatgcactgcaaaccaatcaacccttggtaagcagtcagacaggtttggaatcagtaatgggtaaataccagctactaacttcagttcttcagtgtttgacaaaaatattaaccattgacatggtaatcactgttaagagacaccctcagaaagttcacaatcaagattcagaagatgaactataagcggccgcgtcgac

SEQ ID NO: 34 - DNA, 3467 bp, Artificial sequence
  Construct comprising UBC promoter and COSEQ1-BBS10 nucleotide sequence (referred to as UBC-COSEQ1BBS10)
actagtaacccgtgtcggctccagatctggcctccgcgccgggttttggcgcctcccgcgggcgcccccctcctcacggcgagcgctgccacgtcagacgaagggcgcagcgagcgtcctgatccttccgcccggacgctcaggacagcggcccgctgctcataagactcggccttagaaccccagtatcagcagaaggacattttaggacgggacttgggtgactctagggcactggttttctttccagagagcggaacaggcgaggaaaagtagtcccttctcggcgattctgcggagggatctccgtggggcggtgaacgccgatgattatataaggacgcgccgggtgtggcacagctagttccgtcgcagccgggatttgggtcgcggttcttgtttgtggatcgctgtgatcgtcacttggtgagtagcgggctgctgggctggccggggctttcgtggccgccgggccgctcggtgggacggaagcgtgtggagagaccgccaagggctgtagtctgggtccgcgagcaaggttgccctgaactgggggttggggggagcgcagcaaaatggcggctgttcccgagtcttgaatggaagacgcttgtgaggcgggctgtgaggtcgttgaaacaaggtggggggcatggtgggcggcaagaacccaaggtcttgaggccttcgctaatgcgggaaagctcttattcgggtgagatgggctggggcaccatctggggaccctgacgtgaagtttgtcactgactggagaactcggtttgtcgtctgttgcgggggcggcagttatggcggtgccgttgggcagtgcacccgtacctttgggagcgcgcgccctcgtcgtgtcgtgacgtcacccgttctgttggcttataatgcagggtggggccacctgccggtaggtgtgcggtaggcttttctccgtcgcaggacgcagggttcgggcctagggtaggctctcctgaatcgacaggcgccggacctctggtgaggggagggataagtgaggcgtcagtttctttggtcggttttatgtacctatcttcttaagtagctgaagctccggttttgaactatgcgctcggggttggcgagtgtgttttgtgaagttttttaggcaccttttgaaatgtaatcatttgggtcaatatgtaattttcagtgttagactagtaaattgtccgctaaattctggccgtttttggcttttttgttagacgaagcttgggctgcaggtcgagctcaagcttcgaattcgccaccatgctgtctagcatggctgccgctggatctgtgaaagctgctctgcaggttgccgaggtgctggaagccatcgtgtcttgttgtgtgggacctgagggcagacaggtgctgtgtacaaagcctacaggcgaagtgctgctgagcagaaatggcggcagactgctcgaagccctgcacctggaacaccctatcgccagaatgatcgtggactgcgtgtccagccacctgaagaaaacaggcgacggcgccaagaccttcatcatctttctgtgccatctgctgcggggcctgcacgccatcaccgatagagaaaaggaccctctgatgtgcgagaacatccagacacacggccggcactggaagaactgctcccggtggaagtttatcagccaggctctgctgacctttcagacccagatcctggacggcatcatggaccagtacctgagcagacacttcctgagcatcttcagcagcgccaaagaacggaccctgtgcagaagctctctggaactgctgctcgaggcctacttttgcggcagagtgggcagaaacaaccacaagttcatctcccagctgatgtgtgactacttcttcaagtgcatgacctgcaagagcggcatcggcgtgttcgagctggtggacgatcacttcgtggaactgaatgtgggcgtgaccggcctgcctgtgtccgatagcagaattattgccggcctggtgctgcagaaagacttcagcgtgtacagacccgccgacggcgacatgagaatggtcatcgtgaccgagacaatccagcctctgttcagcacaagcggcagcgagttcatcctgaacagcgaggcccagtttcagaccagccagttctggatcatggaaaagaccaaggccatcatgaagcacctccacagccagaacgtgaagctgctgatctccagcgtgaagcagcccgacctggtgtcttattatgccggcgtgaacggcatcagcgtggtggaatgtctgagcagcgaagaggtgtccctgatcagacggatcatcggactgagcccctttgtgcctcctcaagcctttagccagtgcgagatccctaacacagccctggtcaagttctgcaagcccctgatcctgcggagcaagagatatgtgcacctgggcctgatcagcacatgcgccttcattcctcactccatcgtgctgtgtggacctgtgcacggactgattgagcagcacgaagatgcactgcacggcgccctgaaaatgctgagacagctgttcaaggacctggacctgaactacatgacccagaccaacgaccagaacggcaccagcagcctgttcatctacaagaacagcggcgagagctatcaggccccagatccaggcaatggcagcatccagaggccttaccaggataccgtggccgagaacaaggacgccctggaaaaaacccagacctacctgaaggtgcacagcaacctggtcatccccgatgtggaactggaaacctacattccctacagcacccctacactgacccctaccgataccttccagaccgtggaaaccctgacctgtctgagcctggaacggaacagactgaccgactactacgagcccctgctgaaaaacaacagcaccgcctatagcacccggggcaacagaatcgagatcagctacgagaacctgcaagtgaccaacatcacccggaagggctccatgctgccagtgtcctgcaagctgcctaatatgggcaccagccagagctacctgtcctcttctatgcctgccggatgtgtgctgcctgtcggcggcaattttgagatcctgctgcactactacctgctgaactacgccaagaagtgccaccagagcgaagagacaatggtgtccatgattatcgccaacgctctgctgggcatccccaaggtgctgtacaagagcaagaccggcaagtacagcttccctcacacctacattagagccgtgcacgccctgcagaccaatcagccactggtttctagccagacaggcctggaaagcgtgatgggaaagtaccagctgctgaccagcgtgctgcagtgcctgaccaagatcctgaccatcgacatggtcatcaccgtgaagcggcaccctcagaaagtgcacaaccaggacagcgaggacgagctgtaggcgccgtcgac

SEQ ID NO: 35 - DNA, 3470 bp, Artificial sequence
  Construct comprising UBC promoter and COSEQ2-BBS10 nucleotide sequence (referred to as UBC-COSEQ2-BBS10)
actagtaacccgtgtcggctccagatctggcctccgcgccgggttttggcgcctcccgcgggcgcccccctcctcacggcgagcgctgccacgtcagacgaagggcgcagcgagcgtcctgatccttccgcccggacgctcaggacagcggcccgctgctcataagactcggccttagaaccccagtatcagcagaaggacattttaggacgggacttgggtgactctagggcactggttttctttccagagagcggaacaggcgaggaaaagtagtcccttctcggcgattctgcggagggatctccgtggggcggtgaacgccgatgattatataaggacgcgccgggtgtggcacagctagttccgtcgcagccgggatttgggtcgcggttcttgtttgtggatcgctgtgatcgtcacttggtgagtagcgggctgctgggctggccggggctttcgtggccgccgggccgctcggtgggacggaagcgtgtggagagaccgccaagggctgtagtctgggtccgcgagcaaggttgccctgaactgggggttggggggagcgcagcaaaatggcggctgttcccgagtcttgaatggaagacgcttgtgaggcgggctgtgaggtcgttgaaacaaggtggggggcatggtgggcggcaagaacccaaggtcttgaggccttcgctaatgcgggaaagctcttattcgggtgagatgggctggggcaccatctggggaccctgacgtgaagtttgtcactgactggagaactcggtttgtcgtctgttgcgggggcggcagttatggcggtgccgttgggcagtgcacccgtacctttgggagcgcgcgccctcgtcgtgtcgtgacgtcacccgttctgttggcttataatgcagggtggggccacctgccggtaggtgtgcggtaggcttttctccgtcgcaggacgcagggttcgggcctagggtaggctctcctgaatcgacaggcgccggacctctggtgaggggagggataagtgaggcgtcagtttctttggtcggttttatgtacctatcttcttaagtagctgaagctccggttttgaactatgcgctcggggttggcgagtgtgttttgtgaagttttttaggcaccttttgaaatgtaatcatttgggtcaatatgtaattttcagtgttagactagtaaattgtccgctaaattctggccgtttttggcttttttgttagacgaagcttgggctgcaggtcgagctcaagcttcgaattcgccaccatgctgagctccatggctgccgccggatctgtgaaagccgccctgcaggtggcagaggtgctggaggcaatcgtgagctgttgcgtgggacctgagggccggcaggtgctgtgcacaaagccaaccggcgaggtgctgctgtctagaaatggcggccggctgctggaggccctgcacctggagcacccaattgcaagaatgatcgtggactgcgtgtctagccacctgaagaagacaggcgatggcgccaagaccttcatcatcttcctgtgccacctgctgaggggcctgcacgccatcacagaccgcgagaaggatcctctgatgtgcgagaacatccagacccacggcaggcactggaagaattgttcccgctggaagttcatctctcaggccctgctgacatttcagacccagatcctggacggcatcatggatcagtatctgagcaggcacttcctgtccatcttttcctctgccaaggagcggaccctgtgcagaagctccctggagctgctgctggaggcctacttctgtggccgggtgggcagaaacaatcacaagtttatcagccagctgatgtgcgactatttctttaagtgcatgacctgtaagtccggcatcggcgtgttcgagctggtggacgatcactttgtggagctgaacgtgggagtgacaggcctgcccgtgtccgactctcgcatcatcgccggcctggtgctgcagaaggatttctccgtgtaccggcctgccgacggcgatatgagaatggtcatcgtgaccgagacaatccagccactgttcagcacctccggctctgagttcatcctgaacagcgaggcccagttccagacatctcagttttggatcatggagaagaccaaggccatcatgaagcacctgcacagccagaacgtgaagctgctgatctctagcgtgaagcagccagacctggtgtcttactatgccggcgtgaatggcatcagcgtggtggagtgtctgtcctctgaggaggtgtccctgatccggagaatcattggcctgtctcccttcgtgccccctcaggcctttagccagtgcgagatccccaacacagccctggtgaagttctgtaagcctctgatcctgaggtccaagcggtacgtgcacctgggcctgatcagcacctgcgcctttatcccacactctatcgtgctgtgcggacctgtgcacggcctgattgagcagcacgaggatgcactgcacggcgccctgaagatgctgaggcagctgttcaaggacctggatctgaattacatgacccagacaaacgaccagaatggcacaagctccctgtttatctacaagaactctggcgagagctatcaggccccagatcccggcaatggcagcattcagcgcccctaccaggacacagtggcagagaacaaggatgccctggagaagacccagacatatctgaaggtgcactccaacctggtcatccctgacgtggagctggagacatacatcccttattctaccccaacactgacccccacagataccttccagacagtggagacactgacctgcctgtccctggagaggaaccgcctgaccgactactatgagcccctgctgaagaacaattccacagcctactctacccggggcaatagaatcgagatcagctatgagaacctgcaggtgacaaatatcaccagaaagggctctatgctgcctgtgagctgcaagctgccaaacatgggcaccagccagtcctacctgtctagctccatgcctgcaggatgcgtgctgcctgtgggcggcaacttcgagatcctgctgcactactatctgctgaattatgccaagaagtgccaccagagcgaggagacaatggtgtccatgatcatcgccaacgccctgctgggcatcccaaaggtgctgtacaagtctaagaccggcaagtacagctttccccacacctatatccgggccgtgcacgccctgcagacaaatcagcctctggtgtctagccagaccggcctggagtccgtgatgggcaagtaccagctgctgacatctgtgctgcagtgtctgacaaagatcctgaccatcgatatggtcatcaccgtgaagagacacccacagaaggtgcacaatcaggacagcgaggatgagctgtaagcggccgcgtcgac

SEQ ID NO: 36 - DNA, 2815 bp, Artificial sequence
  Construct comprising CMV promoter and wild type BBS10 nucleotide sequence (referred to as CMV-WTBBS10)
actagttattaatagtaatcaattacggggtcattagttcatagcccatatatggagttccgcgttacataacttacggtaaatggcccgcctggctgaccgcccaacgacccccgcccattgacgtcaataatgacgtatgttcccatagtaacgccaatagggactttccattgacgtcaatgggtggagtatttacggtaaactgcccacttggcagtacatcaagtgtatcatatgccaagtacgccccctattgacgtcaatgacggtaaatggcccgcctggcattatgcccagtacatgaccttatgggactttcctacttggcagtacatctacgtattagtcatcgctattaccatggtgatgcggttttggcagtacatcaatgggcgtggatagcggtttgactcacggggatttccaagtctccaccccattgacgtcaatgggagtttgttttggcaccaaaatcaacgggactttccaaaatgtcgtaacaactccgccccattgacgcaaatgggcggtaggcgtgtacggtgggaggtctatataagcagagctggtttagtgaaccgtcagatccgctagcgctaccggactcagatctcgaattcgccaccatgttaagttctatggccgctgcagggtctgtgaaggcggcgttgcaggtggccgaggtgctggaagccatcgtgagctgctgcgtggggcccgagggacggcaagttttgtgtacgaagcccactggcgaggtgcttctcagccggaatggaggccgcctcctggaggcgctacacttagagcatcccatagccaggatgatagtggactgtgtttccagtcatctcaaaaaaacaggagatggtgcaaaaacatttattatctttctttgccatttgcttagaggacttcatgcaatcacagacagagaaaaggatcctttgatgtgtgaaaacattcaaacccatggaaggcattggaaaaattgttctcggtggaaatttatttcccaggctctcctaacgtttcagacacaaatattagacggtattatggaccagtacctaagtagacactttttgtctatcttttcgtctgctaaagagagaacattgtgtaggagctctttagagttgctcttagaagcatacttttgtggaagagtgggaagaaataatcataaatttatttcacagttgatgtgtgactactttttcaagtgtatgacttgtaaaagtgggattggtgtatttgagttagtggatgaccattttgtagagttgaatgttggtgtcactggccttcctgtttcagattccaggatcatagctggtcttgtgcttcagaaagatttttctgtgtaccgcccagcagatggtgacatgcgaatggtgatagtaacagaaaccattcagcctcttttttccacttctggatcagagtttattctaaattcagaagcacagtttcagacatctcaattttggattatggaaaagacaaaagcaataatgaaacatctacatagtcagaatgtaaaattgctcatatctagtgtgaaacaaccagatttagttagttattatgcaggggtgaatggcatatcagtggttgagtgtttatcatcagaagaagtttctcttatccggaggatcattggtctttctccatttgtaccaccacaggccttttcgcagtgtgaaatacctaacactgctttggtgaaattttgtaaacctcttatccttagatccaaaagatatgttcatctaggcttgataagcacatgtgcatttataccacactctatagttctttgtggaccagtgcatggtctcattgaacaacatgaggatgctttacatggagcacttaaaatgcttcggcaattatttaaagaccttgatctaaattacatgacacaaaccaatgaccaaaatggcacttcaagtctttttatttataagaacagtggagaaagttatcaagcaccagatcctggtaatggctcaatacaaaggccttatcaggacacagttgcagagaacaaagatgcattggaaaaaactcaaacatatttaaaagtacattctaatttggtaattccagatgtagaattagaaacatatattccgtattcaacccccacactgacaccaacagatacattccaaacagttgaaacgctgacatgtttgtctttggaaagaaacaggctaactgattattatgaaccattactcaagaacaattccactgcttattcaacaaggggaaatagaatagaaatttcttacgaaaatttacaggtcacaaatattactagaaagggaagcatgttaccagtgagctgtaagttaccgaatatgggtacttcccagagttacctttcctcatctatgccagctggttgtgttttgccagtaggtggtaattttgagatcttgttacattactatcttctcaattatgccaaaaaatgccatcaatcagaagaaaccatggttagtatgataatagctaatgcacttttaggcattcccaaagtcctttataaatctaaaacaggaaagtacagctttccacatacatatataagagctgtccatgcactgcaaaccaatcaacccttggtaagcagtcagacaggtttggaatcagtaatgggtaaataccagctactaacttcagttcttcagtgtttgacaaaaatattaaccattgacatggtaatcactgttaagagacaccctcagaaagttcacaatcaagattcagaagatgaactataagcggccgcgtcgac

SEQ ID NO: 37 - DNA, 2812 bp, Artificial sequence
  Construct comprising CMV promoter and COSEQ1-BBS10 nucleotide sequence (referred to as CMV-COSEQ1-BBS10)
actagttattaatagtaatcaattacggggtcattagttcatagcccatatatggagttccgcgttacataacttacggtaaatggcccgcctggctgaccgcccaacgacccccgcccattgacgtcaataatgacgtatgttcccatagtaacgccaatagggactttccattgacgtcaatgggtggagtatttacggtaaactgcccacttggcagtacatcaagtgtatcatatgccaagtacgccccctattgacgtcaatgacggtaaatggcccgcctggcattatgcccagtacatgaccttatgggactttcctacttggcagtacatctacgtattagtcatcgctattaccatggtgatgcggttttggcagtacatcaatgggcgtggatagcggtttgactcacggggatttccaagtctccaccccattgacgtcaatgggagtttgttttggcaccaaaatcaacgggactttccaaaatgtcgtaacaactccgccccattgacgcaaatgggcggtaggcgtgtacggtgggaggtctatataagcagagctggtttagtgaaccgtcagatccgctagcgctaccggactcagatctcgaattcgccaccatgctgtctagcatggctgccgctggatctgtgaaagctgctctgcaggttgccgaggtgctggaagccatcgtgtcttgttgtgtgggacctgagggcagacaggtgctgtgtacaaagcctacaggcgaagtgctgctgagcagaaatggcggcagactgctcgaagccctgcacctggaacaccctatcgccagaatgatcgtggactgcgtgtccagccacctgaagaaaacaggcgacggcgccaagaccttcatcatctttctgtgccatctgctgcggggcctgcacgccatcaccgatagagaaaaggaccctctgatgtgcgagaacatccagacacacggccggcactggaagaactgctcccggtggaagtttatcagccaggctctgctgacctttcagacccagatcctggacggcatcatggaccagtacctgagcagacacttcctgagcatcttcagcagcgccaaagaacggaccctgtgcagaagctctctggaactgctgctcgaggcctacttttgcggcagagtgggcagaaacaaccacaagttcatctcccagctgatgtgtgactacttcttcaagtgcatgacctgcaagagcggcatcggcgtgttcgagctggtggacgatcacttcgtggaactgaatgtgggcgtgaccggcctgcctgtgtccgatagcagaattattgccggcctggtgctgcagaaagacttcagcgtgtacagacccgccgacggcgacatgagaatggtcatcgtgaccgagacaatccagcctctgttcagcacaagcggcagcgagttcatcctgaacagcgaggcccagtttcagaccagccagttctggatcatggaaaagaccaaggccatcatgaagcacctccacagccagaacgtgaagctgctgatctccagcgtgaagcagcccgacctggtgtcttattatgccggcgtgaacggcatcagcgtggtggaatgtctgagcagcgaagaggtgtccctgatcagacggatcatcggactgagcccctttgtgcctcctcaagcctttagccagtgcgagatccctaacacagccctggtcaagttctgcaagcccctgatcctgcggagcaagagatatgtgcacctgggcctgatcagcacatgcgccttcattcctcactccatcgtgctgtgtggacctgtgcacggactgattgagcagcacgaagatgcactgcacggcgccctgaaaatgctgagacagctgttcaaggacctggacctgaactacatgacccagaccaacgaccagaacggcaccagcagcctgttcatctacaagaacagcggcgagagctatcaggccccagatccaggcaatggcagcatccagaggccttaccaggataccgtggccgagaacaaggacgccctggaaaaaacccagacctacctgaaggtgcacagcaacctggtcatccccgatgtggaactggaaacctacattccctacagcacccctacactgacccctaccgataccttccagaccgtggaaaccctgacctgtctgagcctggaacggaacagactgaccgactactacgagcccctgctgaaaaacaacagcaccgcctatagcacccggggcaacagaatcgagatcagctacgagaacctgcaagtgaccaacatcacccggaagggctccatgctgccagtgtcctgcaagctgcctaatatgggcaccagccagagctacctgtcctcttctatgcctgccggatgtgtgctgcctgtcggcggcaattttgagatcctgctgcactactacctgctgaactacgccaagaagtgccaccagagcgaagagacaatggtgtccatgattatcgccaacgctctgctgggcatccccaaggtgctgtacaagagcaagaccggcaagtacagcttccctcacacctacattagagccgtgcacgccctgcagaccaatcagccactggtttctagccagacaggcctggaaagcgtgatgggaaagtaccagctgctgaccagcgtgctgcagtgcctgaccaagatcctgaccatcgacatggtcatcaccgtgaagcggcaccctcagaaagtgcacaaccaggacagcgaggacgagctgtaggcgccgtcgac

SEQ ID NO: 38 - DNA, 2815 bp, Artificial sequence
  Construct comprising CMV promoter and COSEQ2-BBS10 nucleotide sequence (referred to as CMV-COSEQ2-BBS10)
actagttattaatagtaatcaattacggggtcattagttcatagcccatatatggagttccgcgttacataacttacggtaaatggcccgcctggctgaccgcccaacgacccccgcccattgacgtcaataatgacgtatgttcccatagtaacgccaatagggactttccattgacgtcaatgggtggagtatttacggtaaactgcccacttggcagtacatcaagtgtatcatatgccaagtacgccccctattgacgtcaatgacggtaaatggcccgcctggcattatgcccagtacatgaccttatgggactttcctacttggcagtacatctacgtattagtcatcgctattaccatggtgatgcggttttggcagtacatcaatgggcgtggatagcggtttgactcacggggatttccaagtctccaccccattgacgtcaatgggagtttgttttggcaccaaaatcaacgggactttccaaaatgtcgtaacaactccgccccattgacgcaaatgggcggtaggcgtgtacggtgggaggtctatataagcagagctggtttagtgaaccgtcagatccgctagcgctaccggactcagatctcgaattcgccaccatgctgagctccatggctgccgccggatctgtgaaagccgccctgcaggtggcagaggtgctggaggcaatcgtgagctgttgcgtgggacctgagggccggcaggtgctgtgcacaaagccaaccggcgaggtgctgctgtctagaaatggcggccggctgctggaggccctgcacctggagcacccaattgcaagaatgatcgtggactgcgtgtctagccacctgaagaagacaggcgatggcgccaagaccttcatcatcttcctgtgccacctgctgaggggcctgcacgccatcacagaccgcgagaaggatcctctgatgtgcgagaacatccagacccacggcaggcactggaagaattgttcccgctggaagttcatctctcaggccctgctgacatttcagacccagatcctggacggcatcatggatcagtatctgagcaggcacttcctgtccatcttttcctctgccaaggagcggaccctgtgcagaagctccctggagctgctgctggaggcctacttctgtggccgggtgggcagaaacaatcacaagtttatcagccagctgatgtgcgactatttctttaagtgcatgacctgtaagtccggcatcggcgtgttcgagctggtggacgatcactttgtggagctgaacgtgggagtgacaggcctgcccgtgtccgactctcgcatcatcgccggcctggtgctgcagaaggatttctccgtgtaccggcctgccgacggcgatatgagaatggtcatcgtgaccgagacaatccagccactgttcagcacctccggctctgagttcatcctgaacagcgaggcccagttccagacatctcagttttggatcatggagaagaccaaggccatcatgaagcacctgcacagccagaacgtgaagctgctgatctctagcgtgaagcagccagacctggtgtcttactatgccggcgtgaatggcatcagcgtggtggagtgtctgtcctctgaggaggtgtccctgatccggagaatcattggcctgtctcccttcgtgccccctcaggcctttagccagtgcgagatccccaacacagccctggtgaagttctgtaagcctctgatcctgaggtccaagcggtacgtgcacctgggcctgatcagcacctgcgcctttatcccacactctatcgtgctgtgcggacctgtgcacggcctgattgagcagcacgaggatgcactgcacggcgccctgaagatgctgaggcagctgttcaaggacctggatctgaattacatgacccagacaaacgaccagaatggcacaagctccctgtttatctacaagaactctggcgagagctatcaggccccagatcccggcaatggcagcattcagcgcccctaccaggacacagtggcagagaacaaggatgccctggagaagacccagacatatctgaaggtgcactccaacctggtcatccctgacgtggagctggagacatacatcccttattctaccccaacactgacccccacagataccttccagacagtggagacactgacctgcctgtccctggagaggaaccgcctgaccgactactatgagcccctgctgaagaacaattccacagcctactctacccggggcaatagaatcgagatcagctatgagaacctgcaggtgacaaatatcaccagaaagggctctatgctgcctgtgagctgcaagctgccaaacatgggcaccagccagtcctacctgtctagctccatgcctgcaggatgcgtgctgcctgtgggcggcaacttcgagatcctgctgcactactatctgctgaattatgccaagaagtgccaccagagcgaggagacaatggtgtccatgatcatcgccaacgccctgctgggcatcccaaaggtgctgtacaagtctaagaccggcaagtacagctttccccacacctatatccgggccgtgcacgccctgcagacaaatcagcctctggtgtctagccagaccggcctggagtccgtgatgggcaagtaccagctgctgacatctgtgctgcagtgtctgacaaagatcctgaccatcgatatggtcatcaccgtgaagagacacccacagaaggtgcacaatcaggacagcgaggatgagctgtaagcggccgcgtcgac

SEQ ID NO: 39 - DNA, 2658 bp, Artificial sequence
  Construct comprising CBA promoter and wild type BBS10 nucleotide sequence (referred to as CBA-WTBBS10)
actagtgtacatctacgtattagtcatcgctattaccatggtcgaggtgagccccacgttctgcttcactctccccatctcccccccctccccacccccaattttgtatttatttattttttaattattttgtgcagcgatgggggcggggggggggggggggcgcgcgccaggcggggcggggcggggcgaggggcggggcggggcgaggcggagaggtgcggcggcagccaatcagagcggcgcgctccgaaagtttccttttatggcgaggcggcggcggcggcggccctataaaaagcgaagcgcgcggcgggcgggagtcgctgcgcgctgccttcgccccgtgccccgctccgccgccgcctcgcgccgcccgccccggctctgactgaccgcgttactcccacaggtgagcgggcgggacggcccttctcctccgggctgtaattagcgcttggaattcgccaccatgttaagttctatggccgctgcagggtctgtgaaggcggcgttgcaggtggccgaggtgctggaagccatcgtgagctgctgcgtggggcccgagggacggcaagttttgtgtacgaagcccactggcgaggtgcttctcagccggaatggaggccgcctcctggaggcgctacacttagagcatcccatagccaggatgatagtggactgtgtttccagtcatctcaaaaaaacaggagatggtgcaaaaacatttattatctttctttgccatttgcttagaggacttcatgcaatcacagacagagaaaaggatcctttgatgtgtgaaaacattcaaacccatggaaggcattggaaaaattgttctcggtggaaatttatttcccaggctctcctaacgtttcagacacaaatattagacggtattatggaccagtacctaagtagacactttttgtctatcttttcgtctgctaaagagagaacattgtgtaggagctctttagagttgctcttagaagcatacttttgtggaagagtgggaagaaataatcataaatttatttcacagttgatgtgtgactactttttcaagtgtatgacttgtaaaagtgggattggtgtatttgagttagtggatgaccattttgtagagttgaatgttggtgtcactggccttcctgtttcagattccaggatcatagctggtcttgtgcttcagaaagatttttctgtgtaccgcccagcagatggtgacatgcgaatggtgatagtaacagaaaccattcagcctcttttttccacttctggatcagagtttattctaaattcagaagcacagtttcagacatctcaattttggattatggaaaagacaaaagcaataatgaaacatctacatagtcagaatgtaaaattgctcatatctagtgtgaaacaaccagatttagttagttattatgcaggggtgaatggcatatcagtggttgagtgtttatcatcagaagaagtttctcttatccggaggatcattggtctttctccatttgtaccaccacaggccttttcgcagtgtgaaatacctaacactgctttggtgaaattttgtaaacctcttatccttagatccaaaagatatgttcatctaggcttgataagcacatgtgcatttataccacactctatagttctttgtggaccagtgcatggtctcattgaacaacatgaggatgctttacatggagcacttaaaatgcttcggcaattatttaaagaccttgatctaaattacatgacacaaaccaatgaccaaaatggcacttcaagtctttttatttataagaacagtggagaaagttatcaagcaccagatcctggtaatggctcaatacaaaggccttatcaggacacagttgcagagaacaaagatgcattggaaaaaactcaaacatatttaaaagtacattctaatttggtaattccagatgtagaattagaaacatatattccgtattcaacccccacactgacaccaacagatacattccaaacagttgaaacgctgacatgtttgtctttggaaagaaacaggctaactgattattatgaaccattactcaagaacaattccactgcttattcaacaaggggaaatagaatagaaatttcttacgaaaatttacaggtcacaaatattactagaaagggaagcatgttaccagtgagctgtaagttaccgaatatgggtacttcccagagttacctttcctcatctatgccagctggttgtgttttgccagtaggtggtaattttgagatcttgttacattactatcttctcaattatgccaaaaaatgccatcaatcagaagaaaccatggttagtatgataatagctaatgcacttttaggcattcccaaagtcctttataaatctaaaacaggaaagtacagctttccacatacatatataagagctgtccatgcactgcaaaccaatcaacccttggtaagcagtcagacaggtttggaatcagtaatgggtaaataccagctactaacttcagttcttcagtgtttgacaaaaatattaaccattgacatggtaatcactgttaagagacaccctcagaaagttcacaatcaagattcagaagatgaactataagcggccgcgtcgac

SEQ ID NO: 40 - DNA, 2655 bp, Artificial sequence
  Construct comprising CBA promoter and COSEQ1-BBS10 nucleotide sequence (referred to as CBA-COSEQ1-BBS10)
actagtgtacatctacgtattagtcatcgctattaccatggtcgaggtgagccccacgttctgcttcactctccccatctcccccccctccccacccccaattttgtatttatttattttttaattattttgtgcagcgatgggggcggggggggggggggggcgcgcgccaggcggggcggggcggggcgaggggcggggcggggcgaggcggagaggtgcggcggcagccaatcagagcggcgcgctccgaaagtttccttttatggcgaggcggcggcggcggcggccctataaaaagcgaagcgcgcggcgggcgggagtcgctgcgcgctgccttcgccccgtgccccgctccgccgccgcctcgcgccgcccgccccggctctgactgaccgcgttactcccacaggtgagcgggcgggacggcccttctcctccgggctgtaattagcgcttggaattcgccaccatgctgtctagcatggctgccgctggatctgtgaaagctgctctgcaggttgccgaggtgctggaagccatcgtgtcttgttgtgtgggacctgagggcagacaggtgctgtgtacaaagcctacaggcgaagtgctgctgagcagaaatggcggcagactgctcgaagccctgcacctggaacaccctatcgccagaatgatcgtggactgcgtgtccagccacctgaagaaaacaggcgacggcgccaagaccttcatcatctttctgtgccatctgctgcggggcctgcacgccatcaccgatagagaaaaggaccctctgatgtgcgagaacatccagacacacggccggcactggaagaactgctcccggtggaagtttatcagccaggctctgctgacctttcagacccagatcctggacggcatcatggaccagtacctgagcagacacttcctgagcatcttcagcagcgccaaagaacggaccctgtgcagaagctctctggaactgctgctcgaggcctacttttgcggcagagtgggcagaaacaaccacaagttcatctcccagctgatgtgtgactacttcttcaagtgcatgacctgcaagagcggcatcggcgtgttcgagctggtggacgatcacttcgtggaactgaatgtgggcgtgaccggcctgcctgtgtccgatagcagaattattgccggcctggtgctgcagaaagacttcagcgtgtacagacccgccgacggcgacatgagaatggtcatcgtgaccgagacaatccagcctctgttcagcacaagcggcagcgagttcatcctgaacagcgaggcccagtttcagaccagccagttctggatcatggaaaagaccaaggccatcatgaagcacctccacagccagaacgtgaagctgctgatctccagcgtgaagcagcccgacctggtgtcttattatgccggcgtgaacggcatcagcgtggtggaatgtctgagcagcgaagaggtgtccctgatcagacggatcatcggactgagcccctttgtgcctcctcaagcctttagccagtgcgagatccctaacacagccctggtcaagttctgcaagcccctgatcctgcggagcaagagatatgtgcacctgggcctgatcagcacatgcgccttcattcctcactccatcgtgctgtgtggacctgtgcacggactgattgagcagcacgaagatgcactgcacggcgccctgaaaatgctgagacagctgttcaaggacctggacctgaactacatgacccagaccaacgaccagaacggcaccagcagcctgttcatctacaagaacagcggcgagagctatcaggccccagatccaggcaatggcagcatccagaggccttaccaggataccgtggccgagaacaaggacgccctggaaaaaacccagacctacctgaaggtgcacagcaacctggtcatccccgatgtggaactggaaacctacattccctacagcacccctacactgacccctaccgataccttccagaccgtggaaaccctgacctgtctgagcctggaacggaacagactgaccgactactacgagcccctgctgaaaaacaacagcaccgcctatagcacccggggcaacagaatcgagatcagctacgagaacctgcaagtgaccaacatcacccggaagggctccatgctgccagtgtcctgcaagctgcctaatatgggcaccagccagagctacctgtcctcttctatgcctgccggatgtgtgctgcctgtcggcggcaattttgagatcctgctgcactactacctgctgaactacgccaagaagtgccaccagagcgaagagacaatggtgtccatgattatcgccaacgctctgctgggcatccccaaggtgctgtacaagagcaagaccggcaagtacagcttccctcacacctacattagagccgtgcacgccctgcagaccaatcagccactggtttctagccagacaggcctggaaagcgtgatgggaaagtaccagctgctgaccagcgtgctgcagtgcctgaccaagatcctgaccatcgacatggtcatcaccgtgaagcggcaccctcagaaagtgcacaaccaggacagcgaggacgagctgtaggcgccgtcgac

SEQ ID NO: 41 - DNA, 2658 bp, Artificial sequence
  Construct comprising CBA promoter and COSEQ2-BBS10 nucleotide sequence (referred to as CBA-COSEQ2-BBS10)
actagtgtacatctacgtattagtcatcgctattaccatggtcgaggtgagccccacgttctgcttcactctccccatctcccccccctccccacccccaattttgtatttatttattttttaattattttgtgcagcgatgggggcggggggggggggggggcgcgcgccaggcggggcggggcggggcgaggggcggggcggggcgaggcggagaggtgcggcggcagccaatcagagcggcgcgctccgaaagtttccttttatggcgaggcggcggcggcggcggccctataaaaagcgaagcgcgcggcgggcgggagtcgctgcgcgctgccttcgccccgtgccccgctccgccgccgcctcgcgccgcccgccccggctctgactgaccgcgttactcccacaggtgagcgggcgggacggcccttctcctccgggctgtaattagcgcttggaattcgccaccatgctgagctccatggctgccgccggatctgtgaaagccgccctgcaggtggcagaggtgctggaggcaatcgtgagctgttgcgtgggacctgagggccggcaggtgctgtgcacaaagccaaccggcgaggtgctgctgtctagaaatggcggccggctgctggaggccctgcacctggagcacccaattgcaagaatgatcgtggactgcgtgtctagccacctgaagaagacaggcgatggcgccaagaccttcatcatcttcctgtgccacctgctgaggggcctgcacgccatcacagaccgcgagaaggatcctctgatgtgcgagaacatccagacccacggcaggcactggaagaattgttcccgctggaagttcatctctcaggccctgctgacatttcagacccagatcctggacggcatcatggatcagtatctgagcaggcacttcctgtccatcttttcctctgccaaggagcggaccctgtgcagaagctccctggagctgctgctggaggcctacttctgtggccgggtgggcagaaacaatcacaagtttatcagccagctgatgtgcgactatttctttaagtgcatgacctgtaagtccggcatcggcgtgttcgagctggtggacgatcactttgtggagctgaacgtgggagtgacaggcctgcccgtgtccgactctcgcatcatcgccggcctggtgctgcagaaggatttctccgtgtaccggcctgccgacggcgatatgagaatggtcatcgtgaccgagacaatccagccactgttcagcacctccggctctgagttcatcctgaacagcgaggcccagttccagacatctcagttttggatcatggagaagaccaaggccatcatgaagcacctgcacagccagaacgtgaagctgctgatctctagcgtgaagcagccagacctggtgtcttactatgccggcgtgaatggcatcagcgtggtggagtgtctgtcctctgaggaggtgtccctgatccggagaatcattggcctgtctcccttcgtgccccctcaggcctttagccagtgcgagatccccaacacagccctggtgaagttctgtaagcctctgatcctgaggtccaagcggtacgtgcacctgggcctgatcagcacctgcgcctttatcccacactctatcgtgctgtgcggacctgtgcacggcctgattgagcagcacgaggatgcactgcacggcgccctgaagatgctgaggcagctgttcaaggacctggatctgaattacatgacccagacaaacgaccagaatggcacaagctccctgtttatctacaagaactctggcgagagctatcaggccccagatcccggcaatggcagcattcagcgcccctaccaggacacagtggcagagaacaaggatgccctggagaagacccagacatatctgaaggtgcactccaacctggtcatccctgacgtggagctggagacatacatcccttattctaccccaacactgacccccacagataccttccagacagtggagacactgacctgcctgtccctggagaggaaccgcctgaccgactactatgagcccctgctgaagaacaattccacagcctactctacccggggcaatagaatcgagatcagctatgagaacctgcaggtgacaaatatcaccagaaagggctctatgctgcctgtgagctgcaagctgccaaacatgggcaccagccagtcctacctgtctagctccatgcctgcaggatgcgtgctgcctgtgggcggcaacttcgagatcctgctgcactactatctgctgaattatgccaagaagtgccaccagagcgaggagacaatggtgtccatgatcatcgccaacgccctgctgggcatcccaaaggtgctgtacaagtctaagaccggcaagtacagctttccccacacctatatccgggccgtgcacgccctgcagacaaatcagcctctggtgtctagccagaccggcctggagtccgtgatgggcaagtaccagctgctgacatctgtgctgcagtgtctgacaaagatcctgaccatcgatatggtcatcaccgtgaagagacacccacagaaggtgcacaatcaggacagcgaggatgagctgtaagcggccgcgtcgac

SEQ ID NO: 42 - DNA, 2901 bp, Artificial sequence
  Construct comprising CAG promoter and wild type BBS10 nucleotide sequence (referred to as CAG-WTBBS10)
actagttcctggaggggtggagtcgtgacctaggccattgacgtcaataatgacgtatgttcccatagtaacgccaatagggactttccattgacgtcaatgggtggagtatttacggtaaactgcccacttggcagtacatcaagtgtatcatatgccaagtacgccccctattgacgtcaatgacggtaaatggcccgcctggcattatgcccagtacatgaccttatgggactttcctacttggcagtacatctacgtattagtcatcgctattaccatggtcgaggtgagccccacgttctgcttcactctccccatctcccccccctccccacccccaattttgtatttatttattttttaattattttgtgcagcgatgggggcggggggggggggggggcgcgcgccaggcggggcggggcggggcgaggggcggggcggggcgaggcggagaggtgcggcggcagccaatcagagcggcgcgctccgaaagtttccttttatggcgaggcggcggcggcggcggccctataaaaagcgaagcgcgcggcgggcgggagtcgctgcgcgctgccttcgccccgtgccccgctccgccgccgcctcgcgccgcccgccccggctctgactgaccgcgttactcccacaggtgagcgggcgggacggcccttctcctccgggctgtaattagcgcttggaattcgccaccatgttaagttctatggccgctgcagggtctgtgaaggcggcgttgcaggtggccgaggtgctggaagccatcgtgagctgctgcgtggggcccgagggacggcaagttttgtgtacgaagcccactggcgaggtgcttctcagccggaatggaggccgcctcctggaggcgctacacttagagcatcccatagccaggatgatagtggactgtgtttccagtcatctcaaaaaaacaggagatggtgcaaaaacatttattatctttctttgccatttgcttagaggacttcatgcaatcacagacagagaaaaggatcctttgatgtgtgaaaacattcaaacccatggaaggcattggaaaaattgttctcggtggaaatttatttcccaggctctcctaacgtttcagacacaaatattagacggtattatggaccagtacctaagtagacactttttgtctatcttttcgtctgctaaagagagaacattgtgtaggagctctttagagttgctcttagaagcatacttttgtggaagagtgggaagaaataatcataaatttatttcacagttgatgtgtgactactttttcaagtgtatgacttgtaaaagtgggattggtgtatttgagttagtggatgaccattttgtagagttgaatgttggtgtcactggccttcctgtttcagattccaggatcatagctggtcttgtgcttcagaaagatttttctgtgtaccgcccagcagatggtgacatgcgaatggtgatagtaacagaaaccattcagcctcttttttccacttctggatcagagtttattctaaattcagaagcacagtttcagacatctcaattttggattatggaaaagacaaaagcaataatgaaacatctacatagtcagaatgtaaaattgctcatatctagtgtgaaacaaccagatttagttagttattatgcaggggtgaatggcatatcagtggttgagtgtttatcatcagaagaagtttctcttatccggaggatcattggtctttctccatttgtaccaccacaggccttttcgcagtgtgaaatacctaacactgctttggtgaaattttgtaaacctcttatccttagatccaaaagatatgttcatctaggcttgataagcacatgtgcatttataccacactctatagttctttgtggaccagtgcatggtctcattgaacaacatgaggatgctttacatggagcacttaaaatgcttcggcaattatttaaagaccttgatctaaattacatgacacaaaccaatgaccaaaatggcacttcaagtctttttatttataagaacagtggagaaagttatcaagcaccagatcctggtaatggctcaatacaaaggccttatcaggacacagttgcagagaacaaagatgcattggaaaaaactcaaacatatttaaaagtacattctaatttggtaattccagatgtagaattagaaacatatattccgtattcaacccccacactgacaccaacagatacattccaaacagttgaaacgctgacatgtttgtctttggaaagaaacaggctaactgattattatgaaccattactcaagaacaattccactgcttattcaacaaggggaaatagaatagaaatttcttacgaaaatttacaggtcacaaatattactagaaagggaagcatgttaccagtgagctgtaagttaccgaatatgggtacttcccagagttacctttcctcatctatgccagctggttgtgttttgccagtaggtggtaattttgagatcttgttacattactatcttctcaattatgccaaaaaatgccatcaatcagaagaaaccatggttagtatgataatagctaatgcacttttaggcattcccaaagtcctttataaatctaaaacaggaaagtacagctttccacatacatatataagagctgtccatgcactgcaaaccaatcaacccttggtaagcagtcagacaggtttggaatcagtaatgggtaaataccagctactaacttcagttcttcagtgtttgacaaaaatattaaccattgacatggtaatcactgttaagagacaccctcagaaagttcacaatcaagattcagaagatgaactataagcggccgcgtcgac

SEQ ID NO: 43 - DNA, 2898 bp, Artificial sequence
  Construct comprising CAG promoter and COSEQ1-BBS10 nucleotide sequence (referred to as CAG-COSEQ1-BBS10)
actagttcctggaggggtggagtcgtgacctaggccattgacgtcaataatgacgtatgttcccatagtaacgccaatagggactttccattgacgtcaatgggtggagtatttacggtaaactgcccacttggcagtacatcaagtgtatcatatgccaagtacgccccctattgacgtcaatgacggtaaatggcccgcctggcattatgcccagtacatgaccttatgggactttcctacttggcagtacatctacgtattagtcatcgctattaccatggtcgaggtgagccccacgttctgcttcactctccccatctcccccccctccccacccccaattttgtatttatttattttttaattattttgtgcagcgatgggggcggggggggggggggggcgcgcgccaggcggggcggggcggggcgaggggcggggcggggcgaggcggagaggtgcggcggcagccaatcagagcggcgcgctccgaaagtttccttttatggcgaggcggcggcggcggcggccctataaaaagcgaagcgcgcggcgggcgggagtcgctgcgcgctgccttcgccccgtgccccgctccgccgccgcctcgcgccgcccgccccggctctgactgaccgcgttactcccacaggtgagcgggcgggacggcccttctcctccgggctgtaattagcgcttggaattcgccaccatgctgtctagcatggctgccgctggatctgtgaaagctgctctgcaggttgccgaggtgctggaagccatcgtgtcttgttgtgtgggacctgagggcagacaggtgctgtgtacaaagcctacaggcgaagtgctgctgagcagaaatggcggcagactgctcgaagccctgcacctggaacaccctatcgccagaatgatcgtggactgcgtgtccagccacctgaagaaaacaggcgacggcgccaagaccttcatcatctttctgtgccatctgctgcggggcctgcacgccatcaccgatagagaaaaggaccctctgatgtgcgagaacatccagacacacggccggcactggaagaactgctcccggtggaagtttatcagccaggctctgctgacctttcagacccagatcctggacggcatcatggaccagtacctgagcagacacttcctgagcatcttcagcagcgccaaagaacggaccctgtgcagaagctctctggaactgctgctcgaggcctacttttgcggcagagtgggcagaaacaaccacaagttcatctcccagctgatgtgtgactacttcttcaagtgcatgacctgcaagagcggcatcggcgtgttcgagctggtggacgatcacttcgtggaactgaatgtgggcgtgaccggcctgcctgtgtccgatagcagaattattgccggcctggtgctgcagaaagacttcagcgtgtacagacccgccgacggcgacatgagaatggtcatcgtgaccgagacaatccagcctctgttcagcacaagcggcagcgagttcatcctgaacagcgaggcccagtttcagaccagccagttctggatcatggaaaagaccaaggccatcatgaagcacctccacagccagaacgtgaagctgctgatctccagcgtgaagcagcccgacctggtgtcttattatgccggcgtgaacggcatcagcgtggtggaatgtctgagcagcgaagaggtgtccctgatcagacggatcatcggactgagcccctttgtgcctcctcaagcctttagccagtgcgagatccctaacacagccctggtcaagttctgcaagcccctgatcctgcggagcaagagatatgtgcacctgggcctgatcagcacatgcgccttcattcctcactccatcgtgctgtgtggacctgtgcacggactgattgagcagcacgaagatgcactgcacggcgccctgaaaatgctgagacagctgttcaaggacctggacctgaactacatgacccagaccaacgaccagaacggcaccagcagcctgttcatctacaagaacagcggcgagagctatcaggccccagatccaggcaatggcagcatccagaggccttaccaggataccgtggccgagaacaaggacgccctggaaaaaacccagacctacctgaaggtgcacagcaacctggtcatccccgatgtggaactggaaacctacattccctacagcacccctacactgacccctaccgataccttccagaccgtggaaaccctgacctgtctgagcctggaacggaacagactgaccgactactacgagcccctgctgaaaaacaacagcaccgcctatagcacccggggcaacagaatcgagatcagctacgagaacctgcaagtgaccaacatcacccggaagggctccatgctgccagtgtcctgcaagctgcctaatatgggcaccagccagagctacctgtcctcttctatgcctgccggatgtgtgctgcctgtcggcggcaattttgagatcctgctgcactactacctgctgaactacgccaagaagtgccaccagagcgaagagacaatggtgtccatgattatcgccaacgctctgctgggcatccccaaggtgctgtacaagagcaagaccggcaagtacagcttccctcacacctacattagagccgtgcacgccctgcagaccaatcagccactggtttctagccagacaggcctggaaagcgtgatgggaaagtaccagctgctgaccagcgtgctgcagtgcctgaccaagatcctgaccatcgacatggtcatcaccgtgaagcggcaccctcagaaagtgcacaaccaggacagcgaggacgagctgtaggcgccgtcgac

SEQ ID NO: 44 - DNA, 2901 bp, Artificial sequence
  Construct comprising CAG promoter and COSEQ2-BBS10 nucleotide sequence (referred to as CAG-COSEQ2-BBS10)
actagttcctggaggggtggagtcgtgacctaggccattgacgtcaataatgacgtatgttcccatagtaacgccaatagggactttccattgacgtcaatgggtggagtatttacggtaaactgcccacttggcagtacatcaagtgtatcatatgccaagtacgccccctattgacgtcaatgacggtaaatggcccgcctggcattatgcccagtacatgaccttatgggactttcctacttggcagtacatctacgtattagtcatcgctattaccatggtcgaggtgagccccacgttctgcttcactctccccatctcccccccctccccacccccaattttgtatttatttattttttaattattttgtgcagcgatgggggcggggggggggggggggcgcgcgccaggcggggcggggcggggcgaggggcggggcggggcgaggcggagaggtgcggcggcagccaatcagagcggcgcgctccgaaagtttccttttatggcgaggcggcggcggcggcggccctataaaaagcgaagcgcgcggcgggcgggagtcgctgcgcgctgccttcgccccgtgccccgctccgccgccgcctcgcgccgcccgccccggctctgactgaccgcgttactcccacaggtgagcgggcgggacggcccttctcctccgggctgtaattagcgcttggaattcgccaccatgctgagctccatggctgccgccggatctgtgaaagccgccctgcaggtggcagaggtgctggaggcaatcgtgagctgttgcgtgggacctgagggccggcaggtgctgtgcacaaagccaaccggcgaggtgctgctgtctagaaatggcggccggctgctggaggccctgcacctggagcacccaattgcaagaatgatcgtggactgcgtgtctagccacctgaagaagacaggcgatggcgccaagaccttcatcatcttcctgtgccacctgctgaggggcctgcacgccatcacagaccgcgagaaggatcctctgatgtgcgagaacatccagacccacggcaggcactggaagaattgttcccgctggaagttcatctctcaggccctgctgacatttcagacccagatcctggacggcatcatggatcagtatctgagcaggcacttcctgtccatcttttcctctgccaaggagcggaccctgtgcagaagctccctggagctgctgctggaggcctacttctgtggccgggtgggcagaaacaatcacaagtttatcagccagctgatgtgcgactatttctttaagtgcatgacctgtaagtccggcatcggcgtgttcgagctggtggacgatcactttgtggagctgaacgtgggagtgacaggcctgcccgtgtccgactctcgcatcatcgccggcctggtgctgcagaaggatttctccgtgtaccggcctgccgacggcgatatgagaatggtcatcgtgaccgagacaatccagccactgttcagcacctccggctctgagttcatcctgaacagcgaggcccagttccagacatctcagttttggatcatggagaagaccaaggccatcatgaagcacctgcacagccagaacgtgaagctgctgatctctagcgtgaagcagccagacctggtgtcttactatgccggcgtgaatggcatcagcgtggtggagtgtctgtcctctgaggaggtgtccctgatccggagaatcattggcctgtctcccttcgtgccccctcaggcctttagccagtgcgagatccccaacacagccctggtgaagttctgtaagcctctgatcctgaggtccaagcggtacgtgcacctgggcctgatcagcacctgcgcctttatcccacactctatcgtgctgtgcggacctgtgcacggcctgattgagcagcacgaggatgcactgcacggcgccctgaagatgctgaggcagctgttcaaggacctggatctgaattacatgacccagacaaacgaccagaatggcacaagctccctgtttatctacaagaactctggcgagagctatcaggccccagatcccggcaatggcagcattcagcgcccctaccaggacacagtggcagagaacaaggatgccctggagaagacccagacatatctgaaggtgcactccaacctggtcatccctgacgtggagctggagacatacatcccttattctaccccaacactgacccccacagataccttccagacagtggagacactgacctgcctgtccctggagaggaaccgcctgaccgactactatgagcccctgctgaagaacaattccacagcctactctacccggggcaatagaatcgagatcagctatgagaacctgcaggtgacaaatatcaccagaaagggctctatgctgcctgtgagctgcaagctgccaaacatgggcaccagccagtcctacctgtctagctccatgcctgcaggatgcgtgctgcctgtgggcggcaacttcgagatcctgctgcactactatctgctgaattatgccaagaagtgccaccagagcgaggagacaatggtgtccatgatcatcgccaacgccctgctgggcatcccaaaggtgctgtacaagtctaagaccggcaagtacagctttccccacacctatatccgggccgtgcacgccctgcagacaaatcagcctctggtgtctagccagaccggcctggagtccgtgatgggcaagtaccagctgctgacatctgtgctgcagtgtctgacaaagatcctgaccatcgatatggtcatcaccgtgaagagacacccacagaaggtgcacaatcaggacagcgaggatgagctgtaagcggccgcgtcgac

SEQ ID NO: 45 - DNA, 204 bp, Human cytomegalovirus
gtgatgcggttttggcagtacatcaatgggcgtggatagcggtttgactcacggggatttccaagtctccaccccattgacgtcaatgggagtttgttttggcaccaaaatcaacgggactttccaaaatgtcgtaacaactccgccccattgacgcaaatgggcggtaggcgtgtacggtgggaggtctatataagcagagct

SEQ ID NO: 46 - DNA, 232 bp, Homo sapiens
ggctccggtgcccgtcagtgggcagagcgcacatcgcccacagtccccgagaagttgtggggaggggtcggcaattgaaccggtgcctagagaaggtggcgcggggtaaactgggaaagtgatgtcgtgtactggctccgcctttttcccgagggtgggggagaaccgtatataagtgcagtagtcgccgtgaacgttctttttcgcaacgggtttgccgccagaacacagg

SEQ ID NO: 47 - DNA, 528 bp, Artificial sequence
  CAG promoter sequence
ccattgacgtcaataatgacgtatgttcccatagtaacgccaatagggactttccattgacgtcaatgggtggagtatttacggtaaactgcccacttggcagtacatcaagtgtatcatatgccaagtacgccccctattgacgtcaatgacggtaaatggcccgcctggcattatgcccagtacatgaccttatgggactttcctacttggcagtacatctacgtattagtcatcgctattaccatggtcgaggtgagccccacgttctgcttcactctccccatctcccccccctccccacccccaattttgtatttatttattttttaattattttgtgcagcgatgggggcggggggggggggggggcgcgcgccaggcggggcggggcggggcgaggggcggggcggggcgaggcggagaggtgcggcggcagccaatcagagcggcgcgctccgaaagtttccttttatggcgaggcggcggcggcggcggccctataaaaagcgaagcgcgcggcgggcg

SEQ ID NO: 48 - DNA, 1170 bp, Homo sapiens
ggcctccgcgccgggttttggcgcctcccgcgggcgcccccctcctcacggcgagcgctgccacgtcagacgaagggcgcagcgagcgtcctgatccttccgcccggacgctcaggacagcggcccgctgctcataagactcggccttagaaccccagtatcagcagaaggacattttaggacgggacttgggtgactctagggcactggttttctttccagagagcggaacaggcgaggaaaagtagtcccttctcggcgattctgcggagggatctccgtggggcggtgaacgccgatgattatataaggacgcgccgggtgtggcacagctagttccgtcgcagccgggatttgggtcgcggttcttgtttgtggatcgctgtgatcgtcacttggtgagtagcgggctgctgggctggccggggctttcgtggccgccgggccgctcggtgggacggaagcgtgtggagagaccgccaagggctgtagtctgggtccgcgagcaaggttgccctgaactgggggttggggggagcgcagcaaaatggcggctgttcccgagtcttgaatggaagacgcttgtgaggcgggctgtgaggtcgttgaaacaaggtggggggcatggtgggcggcaagaacccaaggtcttgaggccttcgctaatgcgggaaagctcttattcgggtgagatgggctggggcaccatctggggaccctgacgtgaagtttgtcactgactggagaactcggtttgtcgtctgttgcgggggcggcagttatggcggtgccgttgggcagtgcacccgtacctttgggagcgcgcgccctcgtcgtgtcgtgacgtcacccgttctgttggcttataatgcagggtggggccacctgccggtaggtgtgcggtaggcttttctccgtcgcaggacgcagggttcgggcctagggtaggctctcctgaatcgacaggcgccggacctctggtgaggggagggataagtgaggcgtcagtttctttggtcggttttatgtacctatcttcttaagtagctgaagctccggttttgaactatgcgctcggggttggcgagtgtgttttgtgaagttttttaggcaccttttgaaatgtaatcatttgggtcaatatgtaattttcagtgttagactagtaaa

SEQ ID NO: 49 - DNA, 278 bp, Gallus gallus
tcgaggtgagccccacgttctgcttcactctccccatctcccccccctccccacccccaattttgtatttatttattttttaattattttgtgcagcgatgggggcggggggggggggggggcgcgcgccaggcggggcggggcggggcgaggggcggggcggggcgaggcggagaggtgcggcggcagccaatcagagcggcgcgctccgaaagtttccttttatggcgaggcggcggcggcggcggccctataaaaagcgaagcgcgcggcgggcg